European Patent Application EP 4 756 024 A1, published June 10, 2026. Title: SIRNA AND COMPOSITION THEREOF. Applicant: Changchun GeneScience Pharmaceuticals Co., Ltd. The sequence listing filed with the application follows.

SEQUENCE LISTING (416 sequences)

SEQ ID NO: 1 - RNA, 23 nt, synthetic construct
  source 1..23: mol_type = other RNA; note = Antisense strand of duplex 1
tagctcactcatgcctcccgcct

SEQ ID NO: 2 - RNA, 23 nt, synthetic construct
  source 1..23: mol_type = other RNA; note = Antisense strand of duplex 2
aatctcttgagatagtcctgagc

SEQ ID NO: 3 - RNA, 23 nt, synthetic construct
  source 1..23: mol_type = other RNA; note = Antisense strand of duplex 3
aaatctcttgagatagtcctgag

SEQ ID NO: 4 - RNA, 23 nt, synthetic construct
  source 1..23: mol_type = other RNA; note = Antisense strand of duplex 4
aaaatctcttgagatagtcctga

SEQ ID NO: 5 - RNA, 23 nt, synthetic construct
  source 1..23: mol_type = other RNA; note = Antisense strand of duplex 5
ataaaatctcttgagatagtcct

SEQ ID NO: 6 - RNA, 23 nt, synthetic construct
  source 1..23: mol_type = other RNA; note = Antisense strand of duplex 6
agataaaatctcttgagatagtc

SEQ ID NO: 7 - RNA, 23 nt, synthetic construct
  source 1..23: mol_type = other RNA; note = Antisense strand of duplex 7
tgtttctgagtcatagagataaa

SEQ ID NO: 8 - RNA, 23 nt, synthetic construct
  source 1..23: mol_type = other RNA; note = Antisense strand of duplex 8
tttgtttctgagtcatagagata

SEQ ID NO: 9 - RNA, 23 nt, synthetic construct
  source 1..23: mol_type = other RNA; note = Antisense strand of duplex 9
ttttgtttctgagtcatagagat

SEQ ID NO: 10 - RNA, 23 nt, synthetic construct
  source 1..23: mol_type = other RNA; note = Antisense strand of duplex 10
agtttggcttctaaactgttggc

SEQ ID NO: 11 - RNA, 23 nt, synthetic construct
  source 1..23: mol_type = other RNA; note = Antisense strand of duplex 11
tgagtttggcttctaaactgttg

SEQ ID NO: 12 - RNA, 23 nt, synthetic construct
  source 1..23: mol_type = other RNA; note = Antisense strand of duplex 12
ttgagtttggcttctaaactgtt

SEQ ID NO: 13 - RNA, 23 nt, synthetic construct
  source 1..23: mol_type = other RNA; note = Antisense strand of duplex 13
acatctccttgagtttggcttct

SEQ ID NO: 14 - RNA, 23 nt, synthetic construct
  source 1..23: mol_type = other RNA; note = Antisense strand of duplex 14
ttaacattccagttataggtagg

SEQ ID NO: 15 - RNA, 23 nt, synthetic construct
  source 1..23: mol_type = other RNA; note = Antisense strand of duplex 15
agtttaacattccagttataggt

SEQ ID NO: 16 - RNA, 23 nt, synthetic construct
  source 1..23: mol_type = other RNA; note = Antisense strand of duplex 16
acatctgggcttctgcattattt

SEQ ID NO: 17 - RNA, 23 nt, synthetic construct
  source 1..23: mol_type = other RNA; note = Antisense strand of duplex 17
tactccacatctgggcttctgca

SEQ ID NO: 18 - RNA, 23 nt, synthetic construct
  source 1..23: mol_type = other RNA; note = Antisense strand of duplex 18
tctggcactccacatctgggctt

SEQ ID NO: 19 - RNA, 23 nt, synthetic construct
  source 1..23: mol_type = other RNA; note = Antisense strand of duplex 19
tatctggcactccacatctgggc

SEQ ID NO: 20 - RNA, 23 nt, synthetic construct
  source 1..23: mol_type = other RNA; note = Antisense strand of duplex 20
tttggaaatagtgagtattctgc

SEQ ID NO: 21 - RNA, 23 nt, synthetic construct
  source 1..23: mol_type = other RNA; note = Antisense strand of duplex 21
atttggaaatagtgagtattctg

SEQ ID NO: 22 - RNA, 23 nt, synthetic construct
  source 1..23: mol_type = other RNA; note = Antisense strand of duplex 22
tatttggaaatagtgagtattct

SEQ ID NO: 23 - RNA, 23 nt, synthetic construct
  source 1..23: mol_type = other RNA; note = Antisense strand of duplex 23
ttatttggaaatagtgagtattc

SEQ ID NO: 24 - RNA, 23 nt, synthetic construct
  source 1..23: mol_type = other RNA; note = Antisense strand of duplex 24
actatttggaaatagtgagtatt

SEQ ID NO: 25 - RNA, 23 nt, synthetic construct
  source 1..23: mol_type = other RNA; note = Antisense strand of duplex 25
ttttgggctatttggaaatagtg

SEQ ID NO: 26 - RNA, 23 nt, synthetic construct
  source 1..23: mol_type = other RNA; note = Antisense strand of duplex 26
tattttgggctatttggaaatag

SEQ ID NO: 27 - RNA, 23 nt, synthetic construct
  source 1..23: mol_type = other RNA; note = Antisense strand of duplex 27
tccattttgggctatttggaaat

SEQ ID NO: 28 - RNA, 23 nt, synthetic construct
  source 1..23: mol_type = other RNA; note = Antisense strand of duplex 28
aagtccattttgggctatttgga

SEQ ID NO: 29 - RNA, 23 nt, synthetic construct
  source 1..23: mol_type = other RNA; note = Antisense strand of duplex 29
tttggaagtccattttgggctat

SEQ ID NO: 30 - RNA, 23 nt, synthetic construct
  source 1..23: mol_type = other RNA; note = Antisense strand of duplex 30
ttttggaagtccattttgggcta

SEQ ID NO: 31 - RNA, 23 nt, synthetic construct
  source 1..23: mol_type = other RNA; note = Antisense strand of duplex 31
actttggaagtccattttgggct

SEQ ID NO: 32 - RNA, 23 nt, synthetic construct
  source 1..23: mol_type = other RNA; note = Antisense strand of duplex 32
agtctcgagtatatgatacgatc

SEQ ID NO: 33 - RNA, 23 nt, synthetic construct
  source 1..23: mol_type = other RNA; note = Antisense strand of duplex 33
taagtctcgagtatatgatacga

SEQ ID NO: 34 - RNA, 23 nt, synthetic construct
  source 1..23: mol_type = other RNA; note = Antisense strand of duplex 34
agtaagtctcgagtatatgatac

SEQ ID NO: 35 - RNA, 23 nt, synthetic construct
  source 1..23: mol_type = other RNA; note = Antisense strand of duplex 35
tgcggtaagtctcgagtatatga

SEQ ID NO: 36 - RNA, 23 nt, synthetic construct
  source 1..23: mol_type = other RNA; note = Antisense strand of duplex 36
atgcggtaagtctcgagtatatg

SEQ ID NO: 37 - RNA, 23 nt, synthetic construct
  source 1..23: mol_type = other RNA; note = Antisense strand of duplex 37
agcctttgacactaatcgatcca

SEQ ID NO: 38 - RNA, 23 nt, synthetic construct
  source 1..23: mol_type = other RNA; note = Antisense strand of duplex 38
aagcctttgacactaatcgatcc

SEQ ID NO: 39 - RNA, 23 nt, synthetic construct
  source 1..23: mol_type = other RNA; note = Antisense strand of duplex 39
aaagcctttgacactaatcgatc

SEQ ID NO: 40 - RNA, 23 nt, synthetic construct
  source 1..23: mol_type = other RNA; note = Antisense strand of duplex 40
taaagcctttgacactaatcgat

SEQ ID NO: 41 - RNA, 23 nt, synthetic construct
  source 1..23: mol_type = other RNA; note = Antisense strand of duplex 41
ttaaagcctttgacactaatcga

SEQ ID NO: 42 - RNA, 23 nt, synthetic construct
  source 1..23: mol_type = other RNA; note = Antisense strand of duplex 42
tttaaagcctttgacactaatcg

SEQ ID NO: 43 - RNA, 23 nt, synthetic construct
  source 1..23: mol_type = other RNA; note = Antisense strand of duplex 43
atttaaagcctttgacactaatc

SEQ ID NO: 44 - RNA, 23 nt, synthetic construct
  source 1..23: mol_type = other RNA; note = Antisense strand of duplex 44
tgtttaaagcctttgacactaat

SEQ ID NO: 45 - RNA, 23 nt, synthetic construct
  source 1..23: mol_type = other RNA; note = Antisense strand of duplex 45
atgtttaaagcctttgacactaa

SEQ ID NO: 46 - RNA, 23 nt, synthetic construct
  source 1..23: mol_type = other RNA; note = Antisense strand of duplex 46
tatgtttaaagcctttgacacta

SEQ ID NO: 47 - RNA, 23 nt, synthetic construct
  source 1..23: mol_type = other RNA; note = Antisense strand of duplex 47
acatgtttaaagcctttgacact

SEQ ID NO: 48 - RNA, 23 nt, synthetic construct
  source 1..23: mol_type = other RNA; note = Antisense strand of duplex 48
tacatgtttaaagcctttgacac

SEQ ID NO: 49 - RNA, 23 nt, synthetic construct
  source 1..23: mol_type = other RNA; note = Antisense strand of duplex 49
tttgccccacatgtttaaagcct

SEQ ID NO: 50 - RNA, 23 nt, synthetic construct
  source 1..23: mol_type = other RNA; note = Antisense strand of duplex 50
agcacggtgagtcgcatagctgc

SEQ ID NO: 51 - RNA, 23 nt, synthetic construct
  source 1..23: mol_type = other RNA; note = Antisense strand of duplex 51
acaactttcctgaaatgcagggg

SEQ ID NO: 52 - RNA, 23 nt, synthetic construct
  source 1..23: mol_type = other RNA; note = Antisense strand of duplex 52
tacaactttcctgaaatgcaggg

SEQ ID NO: 53 - RNA, 23 nt, synthetic construct
  source 1..23: mol_type = other RNA; note = Antisense strand of duplex 53
atacaactttcctgaaatgcagg

SEQ ID NO: 54 - RNA, 23 nt, synthetic construct
  source 1..23: mol_type = other RNA; note = Antisense strand of duplex 54
tatacaactttcctgaaatgcag

SEQ ID NO: 55 - RNA, 23 nt, synthetic construct
  source 1..23: mol_type = other RNA; note = Antisense strand of duplex 55
attccccatacaactttcctgaa

SEQ ID NO: 56 - RNA, 23 nt, synthetic construct
  source 1..23: mol_type = other RNA; note = Antisense strand of duplex 56
agttccccatacaactttcctga

SEQ ID NO: 57 - RNA, 23 nt, synthetic construct
  source 1..23: mol_type = other RNA; note = Antisense strand of duplex 57
tgtcagcagttccccatacaact

SEQ ID NO: 58 - RNA, 23 nt, synthetic construct
  source 1..23: mol_type = other RNA; note = Antisense strand of duplex 58
tcatgatgtcagcagttccccat

SEQ ID NO: 59 - RNA, 23 nt, synthetic construct
  source 1..23: mol_type = other RNA; note = Antisense strand of duplex 59
atcatgatgtcagcagttcccca

SEQ ID NO: 60 - RNA, 23 nt, synthetic construct
  source 1..23: mol_type = other RNA; note = Antisense strand of duplex 60
aatcatgatgtcagcagttcccc

SEQ ID NO: 61 - RNA, 23 nt, synthetic construct
  source 1..23: mol_type = other RNA; note = Antisense strand of duplex 61
tcaatcatgatgtcagcagttcc

SEQ ID NO: 62 - RNA, 23 nt, synthetic construct
  source 1..23: mol_type = other RNA; note = Antisense strand of duplex 62
agccaatcatgatgtcagcagtt

SEQ ID NO: 63 - RNA, 23 nt, synthetic construct
  source 1..23: mol_type = other RNA; note = Antisense strand of duplex 63
aaagccaatcatgatgtcagcag

SEQ ID NO: 64 - RNA, 23 nt, synthetic construct
  source 1..23: mol_type = other RNA; note = Antisense strand of duplex 64
taaagccaatcatgatgtcagca

SEQ ID NO: 65 - RNA, 23 nt, synthetic construct
  source 1..23: mol_type = other RNA; note = Antisense strand of duplex 65
tgcaaagccaatcatgatgtcag

SEQ ID NO: 66 - RNA, 23 nt, synthetic construct
  source 1..23: mol_type = other RNA; note = Antisense strand of duplex 66
acaaaggcatgagccagcgtgtt

SEQ ID NO: 67 - RNA, 23 nt, synthetic construct
  source 1..23: mol_type = other RNA; note = Antisense strand of duplex 67
tgaagtgagcatctcctccgaga

SEQ ID NO: 68 - RNA, 23 nt, synthetic construct
  source 1..23: mol_type = other RNA; note = Antisense strand of duplex 68
tatcctcatcgaagtgagcatct

SEQ ID NO: 69 - RNA, 23 nt, synthetic construct
  source 1..23: mol_type = other RNA; note = Antisense strand of duplex 69
tcatcctcatcgaagtgagcatc

SEQ ID NO: 70 - RNA, 23 nt, synthetic construct
  source 1..23: mol_type = other RNA; note = Antisense strand of duplex 70
ttcatcctcatcgaagtgagcat

SEQ ID NO: 71 - RNA, 23 nt, synthetic construct
  source 1..23: mol_type = other RNA; note = Antisense strand of duplex 71
attcatcctcatcgaagtgagca

SEQ ID NO: 72 - RNA, 23 nt, synthetic construct
  source 1..23: mol_type = other RNA; note = Antisense strand of duplex 72
acgttcatcctcatcgaagtgag

SEQ ID NO: 73 - RNA, 23 nt, synthetic construct
  source 1..23: mol_type = other RNA; note = Antisense strand of duplex 73
tcagcgttcatcctcatcgaagt

SEQ ID NO: 74 - RNA, 23 nt, synthetic construct
  source 1..23: mol_type = other RNA; note = Antisense strand of duplex 74
tccagcgttcatcctcatcgaag

SEQ ID NO: 75 - RNA, 23 nt, synthetic construct
  source 1..23: mol_type = other RNA; note = Antisense strand of duplex 75
tcgtccagcgttcatcctcatcg

SEQ ID NO: 76 - RNA, 23 nt, synthetic construct
  source 1..23: mol_type = other RNA; note = Antisense strand of duplex 76
taccatccgtccagcgttcatcc

SEQ ID NO: 77 - RNA, 23 nt, synthetic construct
  source 1..23: mol_type = other RNA; note = Antisense strand of duplex 77
tgctaccatccgtccagcgttca

SEQ ID NO: 78 - RNA, 23 nt, synthetic construct
  source 1..23: mol_type = other RNA; note = Antisense strand of duplex 78
agactgctaccatccgtccagcg

SEQ ID NO: 79 - RNA, 23 nt, synthetic construct
  source 1..23: mol_type = other RNA; note = Antisense strand of duplex 79
tagactgctaccatccgtccagc

SEQ ID NO: 80 - RNA, 23 nt, synthetic construct
  source 1..23: mol_type = other RNA; note = Antisense strand of duplex 80
ttagactgctaccatccgtccag

SEQ ID NO: 81 - RNA, 23 nt, synthetic construct
  source 1..23: mol_type = other RNA; note = Antisense strand of duplex 81
taaagaatggccaagttcatgag

SEQ ID NO: 82 - RNA, 23 nt, synthetic construct
  source 1..23: mol_type = other RNA; note = Antisense strand of duplex 82
tcaaagaatggccaagttcatga

SEQ ID NO: 83 - RNA, 23 nt, synthetic construct
  source 1..23: mol_type = other RNA; note = Antisense strand of duplex 83
atacccaaagaatggccaagttc

SEQ ID NO: 84 - RNA, 23 nt, synthetic construct
  source 1..23: mol_type = other RNA; note = Antisense strand of duplex 84
tcatacccaaagaatggccaagt

SEQ ID NO: 85 - RNA, 23 nt, synthetic construct
  source 1..23: mol_type = other RNA; note = Antisense strand of duplex 85
tcccatacccaaagaatggccaa

SEQ ID NO: 86 - RNA, 23 nt, synthetic construct
  source 1..23: mol_type = other RNA; note = Antisense strand of duplex 86
atcccatacccaaagaatggcca

SEQ ID NO: 87 - RNA, 23 nt, synthetic construct
  source 1..23: mol_type = other RNA; note = Antisense strand of duplex 87
tgtcccatacccaaagaatggcc

SEQ ID NO: 88 - RNA, 23 nt, synthetic construct
  source 1..23: mol_type = other RNA; note = Antisense strand of duplex 88
atgtcccatacccaaagaatggc

SEQ ID NO: 89 - RNA, 23 nt, synthetic construct
  source 1..23: mol_type = other RNA; note = Antisense strand of duplex 89
aatgtcccatacccaaagaatgg

SEQ ID NO: 90 - RNA, 23 nt, synthetic construct
  source 1..23: mol_type = other RNA; note = Antisense strand of duplex 90
aaatgtcccatacccaaagaatg

SEQ ID NO: 91 - RNA, 23 nt, synthetic construct
  source 1..23: mol_type = other RNA; note = Antisense strand of duplex 91
tttaaaattttggggatctccat

SEQ ID NO: 92 - RNA, 23 nt, synthetic construct
  source 1..23: mol_type = other RNA; note = Antisense strand of duplex 92
atttaaaattttggggatctcca

SEQ ID NO: 93 - RNA, 23 nt, synthetic construct
  source 1..23: mol_type = other RNA; note = Antisense strand of duplex 93
agtttaaaattttggggatctcc

SEQ ID NO: 94 - RNA, 23 nt, synthetic construct
  source 1..23: mol_type = other RNA; note = Antisense strand of duplex 94
aagtttaaaattttggggatctc

SEQ ID NO: 95 - RNA, 23 nt, synthetic construct
  source 1..23: mol_type = other RNA; note = Antisense strand of duplex 95
aaagtttaaaattttggggatct

SEQ ID NO: 96 - RNA, 23 nt, synthetic construct
  source 1..23: mol_type = other RNA; note = Antisense strand of duplex 96
aaaagtttaaaattttggggatc

SEQ ID NO: 97 - RNA, 23 nt, synthetic construct
  source 1..23: mol_type = other RNA; note = Antisense strand of duplex 97
agaaagtttaaaattttggggat

SEQ ID NO: 98 - RNA, 23 nt, synthetic construct
  source 1..23: mol_type = other RNA; note = Antisense strand of duplex 98
tatcctgggaaagtttaaaattt

SEQ ID NO: 99 - RNA, 23 nt, synthetic construct
  source 1..23: mol_type = other RNA; note = Antisense strand of duplex 99
tcatcctgggaaagtttaaaatt

SEQ ID NO: 100 - RNA, 23 nt, synthetic construct
  source 1..23: mol_type = other RNA; note = Antisense strand of duplex 100
atcatcctgggaaagtttaaaat

SEQ ID NO: 101 - RNA, 23 nt, synthetic construct
  source 1..23: mol_type = other RNA; note = Antisense strand of duplex 101
taatatcatcctgggaaagttta

SEQ ID NO: 102 - RNA, 23 nt, synthetic construct
  source 1..23: mol_type = other RNA; note = Antisense strand of duplex 102
ttaatatcatcctgggaaagttt

SEQ ID NO: 103 - RNA, 23 nt, synthetic construct
  source 1..23: mol_type = other RNA; note = Antisense strand of duplex 103
tttaatatcatcctgggaaagtt

SEQ ID NO: 104 - RNA, 23 nt, synthetic construct
  source 1..23: mol_type = other RNA; note = Antisense strand of duplex 104
aaatgcctttaatatcatcctgg

SEQ ID NO: 105 - RNA, 23 nt, synthetic construct
  source 1..23: mol_type = other RNA; note = Antisense strand of duplex 105
tttctgaatgcctttaatatcat

SEQ ID NO: 106 - RNA, 23 nt, synthetic construct
  source 1..23: mol_type = other RNA; note = Antisense strand of duplex 106
atttctgaatgcctttaatatca

SEQ ID NO: 107 - RNA, 23 nt, synthetic construct
  source 1..23: mol_type = other RNA; note = Antisense strand of duplex 107
agtttctgaatgcctttaatatc

SEQ ID NO: 108 - RNA, 23 nt, synthetic construct
  source 1..23: mol_type = other RNA; note = Antisense strand of duplex 108
ttccatatagtttctgaatgcct

SEQ ID NO: 109 - RNA, 23 nt, synthetic construct
  source 1..23: mol_type = other RNA; note = Antisense strand of duplex 109
tttccatatagtttctgaatgcc

SEQ ID NO: 110 - RNA, 23 nt, synthetic construct
  source 1..23: mol_type = other RNA; note = Antisense strand of duplex 110
tctttccatatagtttctgaatg

SEQ ID NO: 111 - RNA, 23 nt, synthetic construct
  source 1..23: mol_type = other RNA; note = Antisense strand of duplex 111
tctctttccatatagtttctgaa

SEQ ID NO: 112 - RNA, 23 nt, synthetic construct
  source 1..23: mol_type = other RNA; note = Antisense strand of duplex 112
attacttctctttccatatagtt

SEQ ID NO: 113 - RNA, 23 nt, synthetic construct
  source 1..23: mol_type = other RNA; note = Antisense strand of duplex 113
tgaattacttctctttccatata

SEQ ID NO: 114 - RNA, 23 nt, synthetic construct
  source 1..23: mol_type = other RNA; note = Antisense strand of duplex 114
tttgaattacttctctttccata

SEQ ID NO: 115 - RNA, 23 nt, synthetic construct
  source 1..23: mol_type = other RNA; note = Antisense strand of duplex 115
tcttgaattacttctctttccat

SEQ ID NO: 116 - RNA, 23 nt, synthetic construct
  source 1..23: mol_type = other RNA; note = Antisense strand of duplex 116
ttcttgaattacttctctttcca

SEQ ID NO: 117 - RNA, 23 nt, synthetic construct
  source 1..23: mol_type = other RNA; note = Antisense strand of duplex 117
tttcttgaattacttctctttcc

SEQ ID NO: 118 - RNA, 23 nt, synthetic construct
  source 1..23: mol_type = other RNA; note = Antisense strand of duplex 118
ttttcttgaattacttctctttc

SEQ ID NO: 119 - RNA, 23 nt, synthetic construct
  source 1..23: mol_type = other RNA; note = Antisense strand of duplex 119
tctttcttgaattacttctcttt

SEQ ID NO: 120 - RNA, 23 nt, synthetic construct
  source 1..23: mol_type = other RNA; note = Antisense strand of duplex 120
ttctttcttgaattacttctctt

SEQ ID NO: 121 - RNA, 23 nt, synthetic construct
  source 1..23: mol_type = other RNA; note = Antisense strand of duplex 121
tttctttcttgaattacttctct

SEQ ID NO: 122 - RNA, 23 nt, synthetic construct
  source 1..23: mol_type = other RNA; note = Antisense strand of duplex 122
atttctttcttgaattacttctc

SEQ ID NO: 123 - RNA, 23 nt, synthetic construct
  source 1..23: mol_type = other RNA; note = Antisense strand of duplex 123
tatttctttcttgaattacttct

SEQ ID NO: 124 - RNA, 23 nt, synthetic construct
  source 1..23: mol_type = other RNA; note = Antisense strand of duplex 124
tctatttctttcttgaattactt

SEQ ID NO: 125 - RNA, 21 nt, synthetic construct
  source 1..21: mol_type = other RNA; note = Sense strand of duplex 1
gcgggaggcatgagtgagcta

SEQ ID NO: 126 - RNA, 21 nt, synthetic construct
  source 1..21: mol_type = other RNA; note = Sense strand of duplex 2
tcaggactatctcaagagatt

SEQ ID NO: 127 - RNA, 21 nt, synthetic construct
  source 1..21: mol_type = other RNA; note = Sense strand of duplex 3
caggactatctcaagagattt

SEQ ID NO: 128 - RNA, 21 nt, synthetic construct
  source 1..21: mol_type = other RNA; note = Sense strand of duplex 4
aggactatctcaagagatttt

SEQ ID NO: 129 - RNA, 21 nt, synthetic construct
  source 1..21: mol_type = other RNA; note = Sense strand of duplex 5
gactatctcaagagattttat

SEQ ID NO: 130 - RNA, 21 nt, synthetic construct
  source 1..21: mol_type = other RNA; note = Sense strand of duplex 6
ctatctcaagagattttatct

SEQ ID NO: 131 - RNA, 21 nt, synthetic construct
  source 1..21: mol_type = other RNA; note = Sense strand of duplex 7
tatctctatgactcagaaaca

SEQ ID NO: 132 - RNA, 21 nt, synthetic construct
  source 1..21: mol_type = other RNA; note = Sense strand of duplex 8
tctctatgactcagaaacaaa

SEQ ID NO: 133 - RNA, 21 nt, synthetic construct
  source 1..21: mol_type = other RNA; note = Sense strand of duplex 9
ctctatgactcagaaacaaaa

SEQ ID NO: 134 - RNA, 21 nt, synthetic construct
  source 1..21: mol_type = other RNA; note = Sense strand of duplex 10
caacagtttagaagccaaact

SEQ ID NO: 135 - RNA, 21 nt, synthetic construct
  source 1..21: mol_type = other RNA; note = Sense strand of duplex 11
acagtttagaagccaaactca

SEQ ID NO: 136 - RNA, 21 nt, synthetic construct
  source 1..21: mol_type = other RNA; note = Sense strand of duplex 12
cagtttagaagccaaactcaa

SEQ ID NO: 137 - RNA, 21 nt, synthetic construct
  source 1..21: mol_type = other RNA; note = Sense strand of duplex 13
aagccaaactcaaggagatgt

SEQ ID NO: 138 - RNA, 21 nt, synthetic construct
  source 1..21: mol_type = other RNA; note = Sense strand of duplex 14
tacctataactggaatgttaa

SEQ ID NO: 139 - RNA, 21 nt, synthetic construct
  source 1..21: mol_type = other RNA; note = Sense strand of duplex 15
ctataactggaatgttaaact

SEQ ID NO: 140 - RNA, 21 nt, synthetic construct
  source 1..21: mol_type = other RNA; note = Sense strand of duplex 16
ataatgcagaagcccagatgt

SEQ ID NO: 141 - RNA, 21 nt, synthetic construct
  source 1..21: mol_type = other RNA; note = Sense strand of duplex 17
cagaagcccagatgtggagta

SEQ ID NO: 142 - RNA, 21 nt, synthetic construct
  source 1..21: mol_type = other RNA; note = Sense strand of duplex 18
gcccagatgtggagtgccaga

SEQ ID NO: 143 - RNA, 21 nt, synthetic construct
  source 1..21: mol_type = other RNA; note = Sense strand of duplex 19
ccagatgtggagtgccagata

SEQ ID NO: 144 - RNA, 21 nt, synthetic construct
  source 1..21: mol_type = other RNA; note = Sense strand of duplex 20
agaatactcactatttccaaa

SEQ ID NO: 145 - RNA, 21 nt, synthetic construct
  source 1..21: mol_type = other RNA; note = Sense strand of duplex 21
gaatactcactatttccaaat

SEQ ID NO: 146 - RNA, 21 nt, synthetic construct
  source 1..21: mol_type = other RNA; note = Sense strand of duplex 22
aatactcactatttccaaata

SEQ ID NO: 147 - RNA, 21 nt, synthetic construct
  source 1..21: mol_type = other RNA; note = Sense strand of duplex 23
atactcactatttccaaataa

SEQ ID NO: 148 - RNA, 21 nt, synthetic construct
  source 1..21: mol_type = other RNA; note = Sense strand of duplex 24
tactcactatttccaaatagt

SEQ ID NO: 149 - RNA, 21 nt, synthetic construct
  source 1..21: mol_type = other RNA; note = Sense strand of duplex 25
ctatttccaaatagcccaaaa

SEQ ID NO: 150 - RNA, 21 nt, synthetic construct
  source 1..21: mol_type = other RNA; note = Sense strand of duplex 26
atttccaaatagcccaaaata

SEQ ID NO: 151 - RNA, 21 nt, synthetic construct
  source 1..21: mol_type = other RNA; note = Sense strand of duplex 27
ttccaaatagcccaaaatgga

SEQ ID NO: 152 - RNA, 21 nt, synthetic construct
  source 1..21: mol_type = other RNA; note = Sense strand of duplex 28
caaatagcccaaaatggactt

SEQ ID NO: 153 - RNA, 21 nt, synthetic construct
  source 1..21: mol_type = other RNA; note = Sense strand of duplex 29
agcccaaaatggacttccaaa

SEQ ID NO: 154 - RNA, 21 nt, synthetic construct
  source 1..21: mol_type = other RNA; note = Sense strand of duplex 30
gcccaaaatggacttccaaaa

SEQ ID NO: 155 - RNA, 21 nt, synthetic construct
  source 1..21: mol_type = other RNA; note = Sense strand of duplex 31
cccaaaatggacttccaaagt

SEQ ID NO: 156 - RNA, 21 nt, synthetic construct
  source 1..21: mol_type = other RNA; note = Sense strand of duplex 32
tcgtatcatatactcgagact

SEQ ID NO: 157 - RNA, 21 nt, synthetic construct
  source 1..21: mol_type = other RNA; note = Sense strand of duplex 33
gtatcatatactcgagactta

SEQ ID NO: 158 - RNA, 21 nt, synthetic construct
  source 1..21: mol_type = other RNA; note = Sense strand of duplex 34
atcatatactcgagacttact

SEQ ID NO: 159 - RNA, 21 nt, synthetic construct
  source 1..21: mol_type = other RNA; note = Sense strand of duplex 35
atatactcgagacttaccgca

SEQ ID NO: 160 - RNA, 21 nt, synthetic construct
  source 1..21: mol_type = other RNA; note = Sense strand of duplex 36
tatactcgagacttaccgcat

SEQ ID NO: 161 - RNA, 21 nt, synthetic construct
  source 1..21: mol_type = other RNA; note = Sense strand of duplex 37
gatcgattagtgtcaaaggct

SEQ ID NO: 162 - RNA, 21 nt, synthetic construct
  source 1..21: mol_type = other RNA; note = Sense strand of duplex 38
atcgattagtgtcaaaggctt

SEQ ID NO: 163 - RNA, 21 nt, synthetic construct
  source 1..21: mol_type = other RNA; note = Sense strand of duplex 39
tcgattagtgtcaaaggcttt

SEQ ID NO: 164 - RNA, 21 nt, synthetic construct
  source 1..21: mol_type = other RNA; note = Sense strand of duplex 40
cgattagtgtcaaaggcttta

SEQ ID NO: 165 - RNA, 21 nt, synthetic construct
  source 1..21: mol_type = other RNA; note = Sense strand of duplex 41
gattagtgtcaaaggctttaa

SEQ ID NO: 166 - RNA, 21 nt, synthetic construct
  source 1..21: mol_type = other RNA; note = Sense strand of duplex 42
attagtgtcaaaggctttaaa

SEQ ID NO: 167 - RNA, 21 nt, synthetic construct
  source 1..21: mol_type = other RNA; note = Sense strand of duplex 43
ttagtgtcaaaggctttaaat

SEQ ID NO: 168 - RNA, 21 nt, synthetic construct
  source 1..21: mol_type = other RNA; note = Sense strand of duplex 44
tagtgtcaaaggctttaaaca

SEQ ID NO: 169 - RNA, 21 nt, synthetic construct
  source 1..21: mol_type = other RNA; note = Sense strand of duplex 45
agtgtcaaaggctttaaacat

SEQ ID NO: 170 - RNA, 21 nt, synthetic construct
  source 1..21: mol_type = other RNA; note = Sense strand of duplex 46
gtgtcaaaggctttaaacata

SEQ ID NO: 171 - RNA, 21 nt, synthetic construct
  source 1..21: mol_type = other RNA; note = Sense strand of duplex 47
tgtcaaaggctttaaacatgt

SEQ ID NO: 172 - RNA, 21 nt, synthetic construct
  source 1..21: mol_type = other RNA; note = Sense strand of duplex 48
gtcaaaggctttaaacatgta

SEQ ID NO: 173 - RNA, 21 nt, synthetic construct
  source 1..21: mol_type = other RNA; note = Sense strand of duplex 49
gctttaaacatgtggggcaaa

SEQ ID NO: 174 - RNA, 21 nt, synthetic construct
  source 1..21: mol_type = other RNA; note = Sense strand of duplex 50
agctatgcgactcaccgtgct

SEQ ID NO: 175 - RNA, 21 nt, synthetic construct
  source 1..21: mol_type = other RNA; note = Sense strand of duplex 51
cctgcatttcaggaaagttgt

SEQ ID NO: 176 - RNA, 21 nt, synthetic construct
  source 1..21: mol_type = other RNA; note = Sense strand of duplex 52
ctgcatttcaggaaagttgta

SEQ ID NO: 177 - RNA, 21 nt, synthetic construct
  source 1..21: mol_type = other RNA; note = Sense strand of duplex 53
tgcatttcaggaaagttgtat

SEQ ID NO: 178 - RNA, 21 nt, synthetic construct
  source 1..21: mol_type = other RNA; note = Sense strand of duplex 54
gcatttcaggaaagttgtata

SEQ ID NO: 179 - RNA, 21 nt, synthetic construct
  source 1..21: mol_type = other RNA; note = Sense strand of duplex 55
caggaaagttgtatggggaat

SEQ ID NO: 180 - RNA, 21 nt, synthetic construct
  source 1..21: mol_type = other RNA; note = Sense strand of duplex 56
aggaaagttgtatggggaact

SEQ ID NO: 181 - RNA, 21 nt, synthetic construct
  source 1..21: mol_type = other RNA; note = Sense strand of duplex 57
ttgtatggggaactgctgaca

SEQ ID NO: 182 - RNA, 21 nt, synthetic construct
  source 1..21: mol_type = other RNA; note = Sense strand of duplex 58
ggggaactgctgacatcatga

SEQ ID NO: 183 - RNA, 21 nt, synthetic construct
  source 1..21: mol_type = other RNA; note = Sense strand of duplex 59
gggaactgctgacatcatgat

SEQ ID NO: 184 - RNA, 21 nt, synthetic construct
  source 1..21: mol_type = other RNA; note = Sense strand of duplex 60
ggaactgctgacatcatgatt

SEQ ID NO: 185 - RNA, 21 nt, synthetic construct
  source 1..21: mol_type = other RNA; note = Sense strand of duplex 61
aactgctgacatcatgattga

SEQ ID NO: 186 - RNA, 21 nt, synthetic construct
  source 1..21: mol_type = other RNA; note = Sense strand of duplex 62
ctgctgacatcatgattggct

SEQ ID NO: 187 - RNA, 21 nt, synthetic construct
  source 1..21: mol_type = other RNA; note = Sense strand of duplex 63
gctgacatcatgattggcttt

SEQ ID NO: 188 - RNA, 21 nt, synthetic construct
  source 1..21: mol_type = other RNA; note = Sense strand of duplex 64
ctgacatcatgattggcttta

SEQ ID NO: 189 - RNA, 21 nt, synthetic construct
  source 1..21: mol_type = other RNA; note = Sense strand of duplex 65
gacatcatgattggctttgca

SEQ ID NO: 190 - RNA, 21 nt, synthetic construct
  source 1..21: mol_type = other RNA; note = Sense strand of duplex 66
cacgctggctcatgcctttgt

SEQ ID NO: 191 - RNA, 21 nt, synthetic construct
  source 1..21: mol_type = other RNA; note = Sense strand of duplex 67
tcggaggagatgctcacttca

SEQ ID NO: 192 - RNA, 21 nt, synthetic construct
  source 1..21: mol_type = other RNA; note = Sense strand of duplex 68
atgctcacttcgatgaggata

SEQ ID NO: 193 - RNA, 21 nt, synthetic construct
  source 1..21: mol_type = other RNA; note = Sense strand of duplex 69
tgctcacttcgatgaggatga

SEQ ID NO: 194 - RNA, 21 nt, synthetic construct
  source 1..21: mol_type = other RNA; note = Sense strand of duplex 70
gctcacttcgatgaggatgaa

SEQ ID NO: 195 - RNA, 21 nt, synthetic construct
  source 1..21: mol_type = other RNA; note = Sense strand of duplex 71
ctcacttcgatgaggatgaat

SEQ ID NO: 196 - RNA, 21 nt, synthetic construct
  source 1..21: mol_type = other RNA; note = Sense strand of duplex 72
cacttcgatgaggatgaacgt

SEQ ID NO: 197 - RNA, 21 nt, synthetic construct
  source 1..21: mol_type = other RNA; note = Sense strand of duplex 73
ttcgatgaggatgaacgctga

SEQ ID NO: 198 - RNA, 21 nt, synthetic construct
  source 1..21: mol_type = other RNA; note = Sense strand of duplex 74
tcgatgaggatgaacgctgga

SEQ ID NO: 199 - RNA, 21 nt, synthetic construct
  source 1..21: mol_type = other RNA; note = Sense strand of duplex 75
atgaggatgaacgctggacga

SEQ ID NO: 200 - RNA, 21 nt, synthetic construct
  source 1..21: mol_type = other RNA; note = Sense strand of duplex 76
atgaacgctggacggatggta

SEQ ID NO: 201 - RNA, 21 nt, synthetic construct
  source 1..21: mol_type = other RNA; note = Sense strand of duplex 77
aacgctggacggatggtagca

SEQ ID NO: 202 - RNA, 21 nt, synthetic construct
  source 1..21: mol_type = other RNA; note = Sense strand of duplex 78
ctggacggatggtagcagtct

SEQ ID NO: 203 - RNA, 21 nt, synthetic construct
  source 1..21: mol_type = other RNA; note = Sense strand of duplex 79
tggacggatggtagcagtcta

SEQ ID NO: 204 - RNA, 21 nt, synthetic construct
  source 1..21: mol_type = other RNA; note = Sense strand of duplex 80
ggacggatggtagcagtctaa

SEQ ID NO: 205 - RNA, 21 nt, synthetic construct
  source 1..21: mol_type = other RNA; note = Sense strand of duplex 81
catgaacttggccattcttta

SEQ ID NO: 206 - RNA, 21 nt, synthetic construct
  source 1..21: mol_type = other RNA; note = Sense strand of duplex 82
atgaacttggccattctttga

SEQ ID NO: 207 - RNA, 21 nt, synthetic construct
  source 1..21: mol_type = other RNA; note = Sense strand of duplex 83
acttggccattctttgggtat

SEQ ID NO: 208 - RNA, 21 nt, synthetic construct
  source 1..21: mol_type = other RNA; note = Sense strand of duplex 84
ttggccattctttgggtatga

SEQ ID NO: 209 - RNA, 21 nt, synthetic construct
  source 1..21: mol_type = other RNA; note = Sense strand of duplex 85
ggccattctttgggtatggga

SEQ ID NO: 210 - RNA, 21 nt, synthetic construct
  source 1..21: mol_type = other RNA; note = Sense strand of duplex 86
gccattctttgggtatgggat

SEQ ID NO: 211 - RNA, 21 nt, synthetic construct
  source 1..21: mol_type = other RNA; note = Sense strand of duplex 87
ccattctttgggtatgggaca

SEQ ID NO: 212 - RNA, 21 nt, synthetic construct
  source 1..21: mol_type = other RNA; note = Sense strand of duplex 88
cattctttgggtatgggacat

SEQ ID NO: 213 - RNA, 21 nt, synthetic construct
  source 1..21: mol_type = other RNA; note = Sense strand of duplex 89
attctttgggtatgggacatt

SEQ ID NO: 214 - RNA, 21 nt, synthetic construct
  source 1..21: mol_type = other RNA; note = Sense strand of duplex 90
ttctttgggtatgggacattt

SEQ ID NO: 215 - RNA, 21 nt, synthetic construct
  source 1..21: mol_type = other RNA; note = Sense strand of duplex 91
ggagatccccaaaattttaaa

SEQ ID NO: 216 - RNA, 21 nt, synthetic construct
  source 1..21: mol_type = other RNA; note = Sense strand of duplex 92
gagatccccaaaattttaaat

SEQ ID NO: 217 - RNA, 21 nt, synthetic construct
  source 1..21: mol_type = other RNA; note = Sense strand of duplex 93
agatccccaaaattttaaact

SEQ ID NO: 218 - RNA, 21 nt, synthetic construct
  source 1..21: mol_type = other RNA; note = Sense strand of duplex 94
gatccccaaaattttaaactt

SEQ ID NO: 219 - RNA, 21 nt, synthetic construct
  source 1..21: mol_type = other RNA; note = Sense strand of duplex 95
atccccaaaattttaaacttt

SEQ ID NO: 220 - RNA, 21 nt, synthetic construct
  source 1..21: mol_type = other RNA; note = Sense strand of duplex 96
tccccaaaattttaaactttt

SEQ ID NO: 221 - RNA, 21 nt, synthetic construct
  source 1..21: mol_type = other RNA; note = Sense strand of duplex 97
ccccaaaattttaaactttct

SEQ ID NO: 222 - RNA, 21 nt, synthetic construct
  source 1..21: mol_type = other RNA; note = Sense strand of duplex 98
attttaaactttcccaggata

SEQ ID NO: 223 - RNA, 21 nt, synthetic construct
  source 1..21: mol_type = other RNA; note = Sense strand of duplex 99
ttttaaactttcccaggatga

SEQ ID NO: 224 - RNA, 21 nt, synthetic construct
  source 1..21: mol_type = other RNA; note = Sense strand of duplex 100
tttaaactttcccaggatgat

SEQ ID NO: 225 - RNA, 21 nt, synthetic construct
  source 1..21: mol_type = other RNA; note = Sense strand of duplex 101
aactttcccaggatgatatta

SEQ ID NO: 226 - RNA, 21 nt, synthetic construct
  source 1..21: mol_type = other RNA; note = Sense strand of duplex 102
actttcccaggatgatattaa

SEQ ID NO: 227 - RNA, 21 nt, synthetic construct
  source 1..21: mol_type = other RNA; note = Sense strand of duplex 103
ctttcccaggatgatattaaa

SEQ ID NO: 228 - RNA, 21 nt, synthetic construct
  source 1..21: mol_type = other RNA; note = Sense strand of duplex 104
aggatgatattaaaggcattt

SEQ ID NO: 229 - RNA, 21 nt, synthetic construct
  source 1..21: mol_type = other RNA; note = Sense strand of duplex 105
gatattaaaggcattcagaaa

SEQ ID NO: 230 - RNA, 21 nt, synthetic construct
  source 1..21: mol_type = other RNA; note = Sense strand of duplex 106
atattaaaggcattcagaaat

SEQ ID NO: 231 - RNA, 21 nt, synthetic construct
  source 1..21: mol_type = other RNA; note = Sense strand of duplex 107
tattaaaggcattcagaaact

SEQ ID NO: 232 - RNA, 21 nt, synthetic construct
  source 1..21: mol_type = other RNA; note = Sense strand of duplex 108
gcattcagaaactatatggaa

SEQ ID NO: 233 - RNA, 21 nt, synthetic construct
  source 1..21: mol_type = other RNA; note = Sense strand of duplex 109
cattcagaaactatatggaaa

SEQ ID NO: 234 - RNA, 21 nt, synthetic construct
  source 1..21: mol_type = other RNA; note = Sense strand of duplex 110
ttcagaaactatatggaaaga

SEQ ID NO: 235 - RNA, 21 nt, synthetic construct
  source 1..21: mol_type = other RNA; note = Sense strand of duplex 111
cagaaactatatggaaagaga

SEQ ID NO: 236 - RNA, 21 nt, synthetic construct
  source 1..21: mol_type = other RNA; note = Sense strand of duplex 112
ctatatggaaagagaagtaat

SEQ ID NO: 237 - RNA, 21 nt, synthetic construct
  source 1..21: mol_type = other RNA; note = Sense strand of duplex 113
tatggaaagagaagtaattca

SEQ ID NO: 238 - RNA, 21 nt, synthetic construct
  source 1..21: mol_type = other RNA; note = Sense strand of duplex 114
tggaaagagaagtaattcaaa

SEQ ID NO: 239 - RNA, 21 nt, synthetic construct
  source 1..21: mol_type = other RNA; note = Sense strand of duplex 115
ggaaagagaagtaattcaaga

SEQ ID NO: 240 - RNA, 21 nt, synthetic construct
  source 1..21: mol_type = other RNA; note = Sense strand of duplex 116
gaaagagaagtaattcaagaa

SEQ ID NO: 241 - RNA, 21 nt, synthetic construct
  source 1..21: mol_type = other RNA; note = Sense strand of duplex 117
aaagagaagtaattcaagaaa

SEQ ID NO: 242 - RNA, 21 nt, synthetic construct
  source 1..21: mol_type = other RNA; note = Sense strand of duplex 118
aagagaagtaattcaagaaaa

SEQ ID NO: 243 - RNA, 21 nt, synthetic construct
  source 1..21: mol_type = other RNA; note = Sense strand of duplex 119
agagaagtaattcaagaaaga

SEQ ID NO: 244 - RNA, 21 nt, synthetic construct
  source 1..21: mol_type = other RNA; note = Sense strand of duplex 120
gagaagtaattcaagaaagaa

SEQ ID NO: 245 - RNA, 21 nt, synthetic construct
  source 1..21: mol_type = other RNA; note = Sense strand of duplex 121
agaagtaattcaagaaagaaa

SEQ ID NO: 246 - RNA, 21 nt, synthetic construct
  source 1..21: mol_type = other RNA; note = Sense strand of duplex 122
gaagtaattcaagaaagaaat

SEQ ID NO: 247 - RNA, 21 nt, synthetic construct
  source 1..21: mol_type = other RNA; note = Sense strand of duplex 123
aagtaattcaagaaagaaata

SEQ ID NO: 248 - RNA, 21 nt, synthetic construct
  source 1..21: mol_type = other RNA; note = Sense strand of duplex 124
gtaattcaagaaagaaataga

SEQ ID NO: 249 - RNA, 23 nt, synthetic construct
  source 1..23: mol_type = other RNA; note = Antisense strand of duplex 125/126
  modified_base order(1,3,4,5,7,10,11,13,15,17,18,19,20,21,22,23): mod_base = OTHER; note = 2'-methoxy modification
  modified_base order(2,6,8,9,12,14,16): mod_base = OTHER; note = 2'-fluorinated
  modified_base order(1^2,2^3,21^22,22^23): mod_base = OTHER; note = Phosphorothioate linkage
aatctcttgagatagtcctgagc

SEQ ID NO: 250 - RNA, 23 nt, synthetic construct
  source 1..23: mol_type = other RNA; note = Antisense strand of duplex 127
  modified_base order(1,3,4,5,6,7,8,10,11,13,15,17,18,19,20,21,22,23): mod_base = OTHER; note = 2'-methoxy modification
  modified_base order(2,9,12,14,16): mod_base = OTHER; note = 2'-fluorinated
  modified_base order(1^2,2^3,21^22,22^23): mod_base = OTHER; note = Phosphorothioate linkage
aatctcttgagatagtcctgagc

SEQ ID NO: 251 - RNA, 23 nt, synthetic construct
  source 1..23: mol_type = other RNA; note = Antisense strand of duplex 128
  modified_base order(1,3,5,6,7,8,9,10,11,13,15,17,18,19,20,21,22,23): mod_base = OTHER; note = 2'-methoxy modification
  modified_base order(2,4,12,14,16): mod_base = OTHER; note = 2'-fluorinated
  modified_base order(1^2,2^3,21^22,22^23): mod_base = OTHER; note = Phosphorothioate linkage
aatctcttgagatagtcctgagc

SEQ ID NO: 252 - RNA, 23 nt, synthetic construct
  source 1..23: mol_type = other RNA; note = Antisense strand of duplex 129/130
  modified_base order(1,3,4,5,7,11,12,13,15,17,18,19,20,21,22,23): mod_base = OTHER; note = 2'-methoxy modification
  modified_base order(2,6,8,9,10,14,16): mod_base = OTHER; note = 2'-fluorinated
  modified_base order(1^2,2^3,21^22,22^23): mod_base = OTHER; note = Phosphorothioate linkage
aatctcttgagatagtcctgagc

SEQ ID NO: 253 - RNA, 23 nt, synthetic construct
  source 1..23: mol_type = other RNA; note = Antisense strand of duplex 131
  modified_base order(1,3,5,7,9,10,11,12,13,15,17,19,21,22,23): mod_base = OTHER; note = 2'-methoxy modification
  modified_base order(2,4,6,8,14,16,18,20): mod_base = OTHER; note = 2'-fluorinated
  modified_base order(1^2,2^3,21^22,22^23): mod_base = OTHER; note = Phosphorothioate linkage
aatctcttgagatagtcctgagc

SEQ ID NO: 254 - RNA, 23 nt, synthetic construct
  source 1..23: mol_type = other RNA; note = Antisense strand of duplex 132
  modified_base order(1,3,4,5,7,8,9,10,11,12,13,15,17,19,20,21,22,23): mod_base = OTHER; note = 2'-methoxy modification
  modified_base order(2,6,14,16,18): mod_base = OTHER; note = 2'-fluorinated
  modified_base order(1^2,2^3,21^22,22^23): mod_base = OTHER; note = Phosphorothioate linkage
aatctcttgagatagtcctgagc

SEQ ID NO: 255 - RNA, 23 nt, synthetic construct
  source 1..23: mol_type = other RNA; note = Antisense strand of duplex 133/134/135/136/137/138/139/140/141/142
  modified_base order(1,3,4,5,6,7,10,11,12,13,15,17,18,19,20,21,22,23): mod_base = OTHER; note = 2'-methoxy modification
  modified_base order(2,8,9,14,16): mod_base = OTHER; note = 2'-fluorinated
  modified_base order(1^2,2^3,21^22,22^23): mod_base = OTHER; note = Phosphorothioate linkage
aatctcttgagatagtcctgagc

SEQ ID NO: 256 - RNA, 23 nt, synthetic construct
  source 1..23: mol_type = other RNA; note = Antisense strand of duplex 143/144/145/146/147/148
  modified_base 1: mod_base = OTHER; note = (E)-vinylphosphonate modification
  modified_base order(1,3,4,5,6,7,10,11,12,13,15,17,18,19,20,21,22,23): mod_base = OTHER; note = 2'-methoxy modification
  modified_base order(2,8,9,14,16): mod_base = OTHER; note = 2'-fluorinated
  modified_base order(1^2,2^3,21^22,22^23): mod_base = OTHER; note = Phosphorothioate linkage
aatctcttgagatagtcctgagc

SEQ ID NO: 257 - RNA, 23 nt, synthetic construct
  source 1..23: mol_type = other RNA; note = Antisense strand of duplex 149/150
  modified_base order(1,3,4,5,7,10,11,13,15,17,18,19,20,21,22,23): mod_base = OTHER; note = 2'-methoxy modification
  modified_base order(2,6,8,9,12,14,16): mod_base = OTHER; note = 2'-fluorinated
  modified_base order(1^2,2^3,21^22,22^23): mod_base = OTHER; note = Phosphorothioate linkage
ttttgtttctgagtcatagagat

SEQ ID NO: 258 - RNA, 23 nt, synthetic construct
  source 1..23: mol_type = other RNA; note = Antisense strand of duplex 151
  modified_base order(1,3,4,5,6,7,8,10,11,13,15,17,18,19,20,21,22,23): mod_base = OTHER; note = 2'-methoxy modification
  modified_base order(2,9,12,14,16): mod_base = OTHER; note = 2'-fluorinated
  modified_base order(1^2,2^3,21^22,22^23): mod_base = OTHER; note = Phosphorothioate linkage
ttttgtttctgagtcatagagat

SEQ ID NO: 259 - RNA, 23 nt, synthetic construct
  source 1..23: mol_type = other RNA; note = Antisense strand of duplex 152
  modified_base order(1,3,5,6,7,8,9,10,11,13,15,17,18,19,20,21,22,23): mod_base = OTHER; note = 2'-methoxy modification
  modified_base order(2,4,12,14,16): mod_base = OTHER; note = 2'-fluorinated
  modified_base order(1^2,2^3,21^22,22^23): mod_base = OTHER; note = Phosphorothioate linkage
ttttgtttctgagtcatagagat

SEQ ID NO: 260 - RNA, 23 nt, synthetic construct
  source 1..23: mol_type = other RNA; note = Antisense strand of duplex 153/154
  modified_base order(1,3,4,5,7,11,12,13,15,17,18,19,20,21,22,23): mod_base = OTHER; note = 2'-methoxy modification
  modified_base order(2,6,8,9,10,14,16): mod_base = OTHER; note = 2'-fluorinated
  modified_base order(1^2,2^3,21^22,22^23): mod_base = OTHER; note = Phosphorothioate linkage
ttttgtttctgagtcatagagat

SEQ ID NO: 261 - RNA, 23 nt, synthetic construct
  source 1..23: mol_type = other RNA; note = Antisense strand of duplex 155
  modified_base order(1,3,5,7,9,10,11,12,13,15,17,19,21,22,23): mod_base = OTHER; note = 2'-methoxy modification
  modified_base order(2,4,6,8,14,16,18,20): mod_base = OTHER; note = 2'-fluorinated
  modified_base order(1^2,2^3,21^22,22^23): mod_base = OTHER; note = Phosphorothioate linkage
ttttgtttctgagtcatagagat

SEQ ID NO: 262 - RNA, 23 nt, synthetic construct
  source 1..23: mol_type = other RNA; note = Antisense strand of duplex 156
  modified_base order(1,3,4,5,7,8,9,10,11,12,13,15,17,19,20,21,22,23): mod_base = OTHER; note = 2'-methoxy modification
  modified_base order(2,6,14,16,18): mod_base = OTHER; note = 2'-fluorinated
  modified_base order(1^2,2^3,21^22,22^23): mod_base = OTHER; note = Phosphorothioate linkage
ttttgtttctgagtcatagagat

SEQ ID NO: 263 - RNA, 23 nt, synthetic construct
  source 1..23: mol_type = other RNA; note = Antisense strand of duplex 157/158/159/160/161/162/163/164/165/166
  modified_base order(1,3,4,5,6,7,10,11,12,13,15,17,18,19,20,21,22,23): mod_base = OTHER; note = 2'-methoxy modification
  modified_base order(2,8,9,14,16): mod_base = OTHER; note = 2'-fluorinated
  modified_base order(1^2,2^3,21^22,22^23): mod_base = OTHER; note = Phosphorothioate linkage
ttttgtttctgagtcatagagat

SEQ ID NO: 264 - RNA, 23 nt, synthetic construct
  source 1..23: mol_type = other RNA; note = Antisense strand of duplex 167/168/169/170/171/172
  modified_base 1: mod_base = OTHER; note = (E)-vinylphosphonate modification
  modified_base order(1,3,4,5,6,7,10,11,12,13,15,17,18,19,20,21,22,23): mod_base = OTHER; note = 2'-methoxy modification
  modified_base order(2,8,9,14,16): mod_base = OTHER; note = 2'-fluorinated
  modified_base order(1^2,2^3,21^22,22^23): mod_base = OTHER; note = Phosphorothioate linkage
ttttgtttctgagtcatagagat

SEQ ID NO: 265 - RNA, 23 nt, synthetic construct
  source 1..23: mol_type = other RNA; note = Antisense strand of duplex 177
  modified_base order(1,3,4,5,7,11,12,13,15,17,18,19,20,21,22,23): mod_base = OTHER; note = 2'-methoxy modification
  modified_base order(2,6,8,9,10,14,16): mod_base = OTHER; note = 2'-fluorinated
  modified_base order(1^2,2^3,21^22,22^23): mod_base = OTHER; note = Phosphorothioate linkage
tgagtttggcttctaaactgttg

SEQ ID NO: 266 - RNA, 23 nt, synthetic construct
  source 1..23: mol_type = other RNA; note = Antisense strand of duplex 180
  modified_base order(1,3,4,5,7,8,9,10,11,12,13,15,17,19,20,21,22,23): mod_base = OTHER; note = 2'-methoxy modification
  modified_base order(2,6,14,16,18): mod_base = OTHER; note = 2'-fluorinated
  modified_base order(1^2,2^3,21^22,22^23): mod_base = OTHER; note = Phosphorothioate linkage
tgagtttggcttctaaactgttg

SEQ ID NO: 267 - RNA, 23 nt, synthetic construct
  source 1..23: mol_type = other RNA; note = Antisense strand of duplex 181/182
  modified_base order(1,3,4,5,6,7,10,11,12,13,15,17,18,19,20,21,22,23): mod_base = OTHER; note = 2'-methoxy modification
  modified_base order(2,8,9,14,16): mod_base = OTHER; note = 2'-fluorinated
  modified_base order(1^2,2^3,21^22,22^23): mod_base = OTHER; note = Phosphorothioate linkage
tgagtttggcttctaaactgttg

SEQ ID NO: 268 - RNA, 23 nt, synthetic construct
  source 1..23: mol_type = other RNA; note = Antisense strand of duplex 183/184
  modified_base order(1,3,4,5,7,10,11,13,15,17,18,19,20,21,22,23): mod_base = OTHER; note = 2'-methoxy modification
  modified_base order(2,6,8,9,12,14,16): mod_base = OTHER; note = 2'-fluorinated
  modified_base order(1^2,2^3,21^22,22^23): mod_base = OTHER; note = Phosphorothioate linkage
ttgagtttggcttctaaactgtt

SEQ ID NO: 269 - RNA, 23 nt, synthetic construct
  source 1..23: mol_type = other RNA; note = Antisense strand of duplex 185
  modified_base order(1,3,4,5,6,7,8,10,11,13,15,17,18,19,20,21,22,23): mod_base = OTHER; note = 2'-methoxy modification
  modified_base order(2,9,12,14,16): mod_base = OTHER; note = 2'-fluorinated
  modified_base order(1^2,2^3,21^22,22^23): mod_base = OTHER; note = Phosphorothioate linkage
ttgagtttggcttctaaactgtt

SEQ ID NO: 270 - RNA, 23 nt, synthetic construct
  source 1..23: mol_type = other RNA; note = Antisense strand of duplex 187
  modified_base order(1,3,4,5,7,11,12,13,15,17,18,19,20,21,22,23): mod_base = OTHER; note = 2'-methoxy modification
  modified_base order(2,6,8,9,10,14,16): mod_base = OTHER; note = 2'-fluorinated
  modified_base order(1^2,2^3,21^22,22^23): mod_base = OTHER; note = Phosphorothioate linkage
ttgagtttggcttctaaactgtt

SEQ ID NO: 271 - RNA, 23 nt, synthetic construct
  source 1..23: mol_type = other RNA; note = Antisense strand of duplex 188/189
  modified_base order(1,3,4,5,7,10,11,13,15,17,18,19,20,21,22,23): mod_base = OTHER; note = 2'-methoxy modification
  modified_base order(2,6,8,9,12,14,16): mod_base = OTHER; note = 2'-fluorinated
  modified_base order(1^2,2^3,21^22,22^23): mod_base = OTHER; note = Phosphorothioate linkage
aagcctttgacactaatcgatcc

SEQ ID NO: 272 - RNA, 23 nt, synthetic construct
  source 1..23: mol_type = other RNA; note = Antisense strand of duplex 190
  modified_base order(1,3,4,5,6,7,8,10,11,13,15,17,18,19,20,21,22,23): mod_base = OTHER; note = 2'-methoxy modification
  modified_base order(2,9,12,14,16): mod_base = OTHER; note = 2'-fluorinated
  modified_base order(1^2,2^3,21^22,22^23): mod_base = OTHER; note = Phosphorothioate linkage
aagcctttgacactaatcgatcc

SEQ ID NO: 273 - RNA, 23 nt, synthetic construct
  source 1..23: mol_type = other RNA; note = Antisense strand of duplex 191
  modified_base order(1,3,5,6,7,8,9,10,11,13,15,17,18,19,20,21,22,23): mod_base = OTHER; note = 2'-methoxy modification
  modified_base order(2,4,12,14,16): mod_base = OTHER; note = 2'-fluorinated
  modified_base order(1^2,2^3,21^22,22^23): mod_base = OTHER; note = Phosphorothioate linkage
aagcctttgacactaatcgatcc

SEQ ID NO: 274 - RNA, 23 nt, synthetic construct
  source 1..23: mol_type = other RNA; note = Antisense strand of duplex 192/193
  modified_base order(1,3,4,5,7,11,12,13,15,17,18,19,20,21,22,23): mod_base = OTHER; note = 2'-methoxy modification
  modified_base order(2,6,8,9,10,14,16): mod_base = OTHER; note = 2'-fluorinated
  modified_base order(1^2,2^3,21^22,22^23): mod_base = OTHER; note = Phosphorothioate linkage
aagcctttgacactaatcgatcc

SEQ ID NO: 275 - RNA, 23 nt, synthetic construct
  source 1..23: mol_type = other RNA; note = Antisense strand of duplex 194
  modified_base order(1,3,5,7,9,11,12,13,15,17,19,21,22,23): mod_base = OTHER; note = 2'-methoxy modification
  modified_base order(2,4,6,8,10,14,16,18,20): mod_base = OTHER; note = 2'-fluorinated
  modified_base order(1^2,2^3,21^22,22^23): mod_base = OTHER; note = Phosphorothioate linkage
aagcctttgacactaatcgatcc

SEQ ID NO: 276 - RNA, 23 nt, synthetic construct
  source 1..23: mol_type = other RNA; note = Antisense strand of duplex 195
  modified_base order(1,3,4,5,7,8,9,10,11,12,13,15,17,19,20,21,22,23): mod_base = OTHER; note = 2'-methoxy modification
  modified_base order(2,6,14,16,18): mod_base = OTHER; note = 2'-fluorinated
  modified_base order(1^2,2^3,21^22,22^23): mod_base = OTHER; note = Phosphorothioate linkage
aagcctttgacactaatcgatcc

SEQ ID NO: 277 - RNA, 23 nt, synthetic construct
  source 1..23: mol_type = other RNA; note = Antisense strand of duplex 196/197
  modified_base order(1,3,4,5,6,7,10,11,12,13,15,17,18,19,20,21,22,23): mod_base = OTHER; note = 2'-methoxy modification
  modified_base order(2,8,9,14,16): mod_base = OTHER; note = 2'-fluorinated
  modified_base order(1^2,2^3,21^22,22^23): mod_base = OTHER; note = Phosphorothioate linkage
aagcctttgacactaatcgatcc

SEQ ID NO: 278 - RNA, 23 nt, synthetic construct
  source 1..23: mol_type = other RNA; note = Antisense strand of duplex 198/199
  modified_base order(1,3,4,5,7,10,11,13,15,17,18,19,20,21,22,23): mod_base = OTHER; note = 2'-methoxy modification
  modified_base order(2,6,8,9,12,14,16): mod_base = OTHER; note = 2'-fluorinated
  modified_base order(1^2,2^3,21^22,22^23): mod_base = OTHER; note = Phosphorothioate linkage
tatgtttaaagcctttgacacta

SEQ ID NO: 279 - RNA, 23 nt, synthetic construct
  source 1..23: mol_type = other RNA; note = Antisense strand of duplex 200
  modified_base order(1,3,4,5,6,7,8,10,11,13,15,17,18,19,20,21,22,23): mod_base = OTHER; note = 2'-methoxy modification
  modified_base order(2,9,12,14,16): mod_base = OTHER; note = 2'-fluorinated
  modified_base order(1^2,2^3,21^22,22^23): mod_base = OTHER; note = Phosphorothioate linkage
tatgtttaaagcctttgacacta

SEQ ID NO: 280 - RNA, 23 nt, synthetic construct
  source 1..23: mol_type = other RNA; note = Antisense strand of duplex 201
  modified_base order(1,3,5,6,7,8,9,10,11,13,15,17,18,19,20,21,22,23): mod_base = OTHER; note = 2'-methoxy modification
  modified_base order(2,4,12,14,16): mod_base = OTHER; note = 2'-fluorinated
  modified_base order(1^2,2^3,21^22,22^23): mod_base = OTHER; note = Phosphorothioate linkage
tatgtttaaagcctttgacacta

SEQ ID NO: 281 - RNA, 23 nt, synthetic construct
  source 1..23: mol_type = other RNA; note = Antisense strand of duplex 202/203
  modified_base order(1,3,4,5,7,11,12,13,15,17,18,19,20,21,22,23): mod_base = OTHER; note = 2'-methoxy modification
  modified_base order(2,6,8,9,10,14,16): mod_base = OTHER; note = 2'-fluorinated
  modified_base order(1^2,2^3,21^22,22^23): mod_base = OTHER; note = Phosphorothioate linkage
tatgtttaaagcctttgacacta

SEQ ID NO: 282 - RNA, 23 nt, synthetic construct
  source 1..23: mol_type = other RNA; note = Antisense strand of duplex 204
  modified_base order(1,3,5,7,9,11,12,13,15,17,19,21,22,23): mod_base = OTHER; note = 2'-methoxy modification
  modified_base order(2,4,6,8,10,14,16,18,20): mod_base = OTHER; note = 2'-fluorinated
  modified_base order(1^2,2^3,21^22,22^23): mod_base = OTHER; note = Phosphorothioate linkage
tatgtttaaagcctttgacacta

SEQ ID NO: 283 - RNA, 23 nt, synthetic construct
  source 1..23: mol_type = other RNA; note = Antisense strand of duplex 205
  modified_base order(1,3,4,5,7,8,9,10,11,12,13,15,17,19,20,21,22,23): mod_base = OTHER; note = 2'-methoxy modification
  modified_base order(2,6,14,16,18): mod_base = OTHER; note = 2'-fluorinated
  modified_base order(1^2,2^3,21^22,22^23): mod_base = OTHER; note = Phosphorothioate linkage
tatgtttaaagcctttgacacta

SEQ ID NO: 284 - RNA, 23 nt, synthetic construct
  source 1..23: mol_type = other RNA; note = Antisense strand of duplex 206/207
  modified_base order(1,3,4,5,6,7,10,11,12,13,15,17,18,19,20,21,22,23): mod_base = OTHER; note = 2'-methoxy modification
  modified_base order(2,8,9,14,16): mod_base = OTHER; note = 2'-fluorinated
  modified_base order(1^2,2^3,21^22,22^23): mod_base = OTHER; note = Phosphorothioate linkage
tatgtttaaagcctttgacacta

SEQ ID NO: 285 - RNA, 23 nt, synthetic construct
  source 1..23: mol_type = other RNA; note = Antisense strand of duplex 208/213
  modified_base 1: mod_base = OTHER; note = (E)-vinylphosphonate modification
  modified_base order(1,3,4,5,7,10,11,13,15,17,18,19,20,21,22,23): mod_base = OTHER; note = 2'-methoxy modification
  modified_base order(2,6,8,9,12,14,16): mod_base = OTHER; note = 2'-fluorinated
  modified_base order(1^2,2^3,21^22,22^23): mod_base = OTHER; note = Phosphorothioate linkage
tatgtttaaagcctttgacacta

SEQ ID NO: 286 - RNA, 23 nt, synthetic construct
  source 1..23: mol_type = other RNA; note = Antisense strand of duplex 209/214
  modified_base 1: mod_base = OTHER; note = (E)-vinylphosphonate modification
  modified_base order(1,3,4,5,6,7,8,10,11,13,15,17,18,19,20,21,22,23): mod_base = OTHER; note = 2'-methoxy modification
  modified_base order(2,9,12,14,16): mod_base = OTHER; note = 2'-fluorinated
  modified_base order(1^2,2^3,21^22,22^23): mod_base = OTHER; note = Phosphorothioate linkage
tatgtttaaagcctttgacacta

SEQ ID NO: 287 - RNA, 23 nt, synthetic construct
  source 1..23: mol_type = other RNA; note = Antisense strand of duplex 210/215
  modified_base 1: mod_base = OTHER; note = (E)-vinylphosphonate modification
  modified_base order(1,3,4,5,7,11,12,13,15,17,18,19,20,21,22,23): mod_base = OTHER; note = 2'-methoxy modification
  modified_base order(2,6,8,9,10,14,16): mod_base = OTHER; note = 2'-fluorinated
  modified_base order(1^2,2^3,21^22,22^23): mod_base = OTHER; note = Phosphorothioate linkage
tatgtttaaagcctttgacacta

SEQ ID NO: 288 - RNA, 23 nt, synthetic construct
  source 1..23: mol_type = other RNA; note = Antisense strand of duplex 211/212/216/217
  modified_base 1: mod_base = OTHER; note = (E)-vinylphosphonate modification
  modified_base order(1,3,4,5,6,7,10,11,12,13,15,17,18,19,20,21,22,23): mod_base = OTHER; note = 2'-methoxy modification
  modified_base order(2,8,9,14,16): mod_base = OTHER; note = 2'-fluorinated
  modified_base order(1^2,2^3,21^22,22^23): mod_base = OTHER; note = Phosphorothioate linkage
tatgtttaaagcctttgacacta

SEQ ID NO: 289 - RNA, 23 nt, synthetic construct
  source 1..23: mol_type = other RNA; note = Antisense strand of duplex 218/219
  modified_base order(1,3,4,5,7,10,11,13,15,17,18,19,20,21,22,23): mod_base = OTHER; note = 2'-methoxy modification
  modified_base order(2,6,8,9,12,14,16): mod_base = OTHER; note = 2'-fluorinated
  modified_base order(1^2,2^3,21^22,22^23): mod_base = OTHER; note = Phosphorothioate linkage
tgaagtgagcatctcctccgaga

SEQ ID NO: 290 - RNA, 23 nt, synthetic construct
  source 1..23: mol_type = other RNA; note = Antisense strand of duplex 220
  modified_base order(1,3,4,5,6,7,8,10,11,13,15,17,18,19,20,21,22,23): mod_base = OTHER; note = 2'-methoxy modification
  modified_base order(2,9,12,14,16): mod_base = OTHER; note = 2'-fluorinated
  modified_base order(1^2,2^3,21^22,22^23): mod_base = OTHER; note = Phosphorothioate linkage
tgaagtgagcatctcctccgaga

SEQ ID NO: 291 - RNA, 23 nt, synthetic construct
  source 1..23: mol_type = other RNA; note = Antisense strand of duplex 221
  modified_base order(1,3,5,6,7,8,9,10,11,13,15,17,18,19,20,21,22,23): mod_base = OTHER; note = 2'-methoxy modification
  modified_base order(2,4,12,14,16): mod_base = OTHER; note = 2'-fluorinated
  modified_base order(1^2,2^3,21^22,22^23): mod_base = OTHER; note = Phosphorothioate linkage
tgaagtgagcatctcctccgaga

SEQ ID NO: 292 - RNA, 23 nt, synthetic construct
  source 1..23: mol_type = other RNA; note = Antisense strand of duplex 222/223
  modified_base order(1,3,4,5,7,11,12,13,15,17,18,19,20,21,22,23): mod_base = OTHER; note = 2'-methoxy modification
  modified_base order(2,6,8,9,10,14,16): mod_base = OTHER; note = 2'-fluorinated
  modified_base order(1^2,2^3,21^22,22^23): mod_base = OTHER; note = Phosphorothioate linkage
tgaagtgagcatctcctccgaga

SEQ ID NO: 293 - RNA, 23 nt, synthetic construct
  source 1..23: mol_type = other RNA; note = Antisense strand of duplex 224
  modified_base order(1,3,5,7,9,11,12,13,15,17,19,21,22,23): mod_base = OTHER; note = 2'-methoxy modification
  modified_base order(2,4,6,8,10,14,16,18,20): mod_base = OTHER; note = 2'-fluorinated
  modified_base order(1^2,2^3,21^22,22^23): mod_base = OTHER; note = Phosphorothioate linkage
tgaagtgagcatctcctccgaga

SEQ ID NO: 294 - RNA, 23 nt, synthetic construct
  source 1..23: mol_type = other RNA; note = Antisense strand of duplex 225
  modified_base order(1,3,4,5,7,8,9,10,11,12,13,15,17,19,20,21,22,23): mod_base = OTHER; note = 2'-methoxy modification
  modified_base order(2,6,14,16,18): mod_base = OTHER; note = 2'-fluorinated
  modified_base order(1^2,2^3,21^22,22^23): mod_base = OTHER; note = Phosphorothioate linkage
tgaagtgagcatctcctccgaga

SEQ ID NO: 295 - RNA, 23 nt, synthetic construct
  source 1..23: mol_type = other RNA; note = Antisense strand of duplex 226/227
  modified_base order(1,3,4,5,6,7,10,11,12,13,15,17,18,19,20,21,22,23): mod_base = OTHER; note = 2'-methoxy modification
  modified_base order(2,8,9,14,16): mod_base = OTHER; note = 2'-fluorinated
  modified_base order(1^2,2^3,21^22,22^23): mod_base = OTHER; note = Phosphorothioate linkage
tgaagtgagcatctcctccgaga

SEQ ID NO: 296 - RNA, 23 nt, synthetic construct
  source 1..23: mol_type = other RNA; note = Antisense strand of duplex 228/229
  modified_base order(1,3,4,5,7,10,11,13,15,17,18,19,20,21,22,23): mod_base = OTHER; note = 2'-methoxy modification
  modified_base order(2,6,8,9,12,14,16): mod_base = OTHER; note = 2'-fluorinated
  modified_base order(1^2,2^3,21^22,22^23): mod_base = OTHER; note = Phosphorothioate linkage
tcagcgttcatcctcatcgaagt

SEQ ID NO: 297 - RNA, 23 nt, synthetic construct
  source 1..23: mol_type = other RNA; note = Antisense strand of duplex 230
  modified_base order(1,3,4,5,6,7,8,10,11,13,15,17,18,19,20,21,22,23): mod_base = OTHER; note = 2'-methoxy modification
  modified_base order(2,9,12,14,16): mod_base = OTHER; note = 2'-fluorinated
  modified_base order(1^2,2^3,21^22,22^23): mod_base = OTHER; note = Phosphorothioate linkage
tcagcgttcatcctcatcgaagt

SEQ ID NO: 298 - RNA, 23 nt, synthetic construct
  source 1..23: mol_type = other RNA; note = Antisense strand of duplex 231
  modified_base order(1,3,5,6,7,8,9,10,11,13,15,17,18,19,20,21,22,23): mod_base = OTHER; note = 2'-methoxy modification
  modified_base order(2,4,12,14,16): mod_base = OTHER; note = 2'-fluorinated
  modified_base order(1^2,2^3,21^22,22^23): mod_base = OTHER; note = Phosphorothioate linkage
tcagcgttcatcctcatcgaagt

SEQ ID NO: 299 - RNA, 23 nt, synthetic construct
  source 1..23: mol_type = other RNA; note = Antisense strand of duplex 232/233
  modified_base order(1,3,4,5,7,11,12,13,15,17,18,19,20,21,22,23): mod_base = OTHER; note = 2'-methoxy modification
  modified_base order(2,6,8,9,10,14,16): mod_base = OTHER; note = 2'-fluorinated
  modified_base order(1^2,2^3,21^22,22^23): mod_base = OTHER; note = Phosphorothioate linkage
tcagcgttcatcctcatcgaagt

SEQ ID NO: 300 - RNA, 23 nt, synthetic construct
  source 1..23: mol_type = other RNA; note = Antisense strand of duplex 234
  modified_base order(1,3,5,7,9,11,12,13,15,17,19,21,22,23): mod_base = OTHER; note = 2'-methoxy modification
  modified_base order(2,4,6,8,10,14,16,18,20): mod_base = OTHER; note = 2'-fluorinated
  modified_base order(1^2,2^3,21^22,22^23): mod_base = OTHER; note = Phosphorothioate linkage
tcagcgttcatcctcatcgaagt

SEQ ID NO: 301 - RNA, 23 nt, synthetic construct
  source 1..23: mol_type = other RNA; note = Antisense strand of duplex 235
  modified_base order(1,3,4,5,7,8,9,10,11,12,13,15,17,19,20,21,22,23): mod_base = OTHER; note = 2'-methoxy modification
  modified_base order(2,6,14,16,18): mod_base = OTHER; note = 2'-fluorinated
  modified_base order(1^2,2^3,21^22,22^23): mod_base = OTHER; note = Phosphorothioate linkage
tcagcgttcatcctcatcgaagt

SEQ ID NO: 302 - RNA, 23 nt, synthetic construct
  source 1..23: mol_type = other RNA; note = Antisense strand of duplex 236/237
  modified_base order(1,3,4,5,6,7,10,11,12,13,15,17,18,19,20,21,22,23): mod_base = OTHER; note = 2'-methoxy modification
  modified_base order(2,8,9,14,16): mod_base = OTHER; note = 2'-fluorinated
  modified_base order(1^2,2^3,21^22,22^23): mod_base = OTHER; note = Phosphorothioate linkage
tcagcgttcatcctcatcgaagt

SEQ ID NO: 303 - RNA, 21 nt, synthetic construct
  source 1..21: mol_type = other RNA; note = Sense strand of duplex 125/128
  modified_base order(1,2,3,4,5,6,8,10,12,13,14,15,16,17,18,19,20,21): mod_base = OTHER; note = 2'-methoxy modification
  modified_base order(7,9,11): mod_base = OTHER; note = 2'-fluorinated
  modified_base order(1^2,2^3): mod_base = OTHER; note = Phosphorothioate linkage
tcaggactatctcaagagatt

SEQ ID NO: 304 - RNA, 21 nt, synthetic construct
  source 1..21: mol_type = other RNA; note = Sense strand of duplex 126/127
  modified_base order(1,2,3,4,5,6,7,8,10,12,14,15,16,17,18,19,20,21): mod_base = OTHER; note = 2'-methoxy modification
  modified_base order(9,11,13): mod_base = OTHER; note = 2'-fluorinated
  modified_base order(1^2,2^3): mod_base = OTHER; note = Phosphorothioate linkage
tcaggactatctcaagagatt

SEQ ID NO: 305 - RNA, 21 nt, synthetic construct
  source 1..21: mol_type = other RNA; note = Sense strand of duplex 129
  modified_base order(1,2,3,4,5,6,8,12,13,14,16,17,18,19,20,21): mod_base = OTHER; note = 2'-methoxy modification
  modified_base order(7,9,10,11,15): mod_base = OTHER; note = 2'-fluorinated
  modified_base order(1^2,2^3): mod_base = OTHER; note = Phosphorothioate linkage
tcaggactatctcaagagatt

SEQ ID NO: 306 - RNA, 21 nt, synthetic construct
  source 1..21: mol_type = other RNA; note = Sense strand of duplex 130/131
  modified_base order(1,2,3,4,5,6,8,12,13,14,15,16,17,18,19,20,21): mod_base = OTHER; note = 2'-methoxy modification
  modified_base order(7,9,10): mod_base = OTHER; note = 2'-fluorinated
  modified_base 11: mod_base = OTHER; note = Deoxynucleotide
  modified_base order(1^2,2^3): mod_base = OTHER; note = Phosphorothioate linkage
tcaggactatctcaagagatt

SEQ ID NO: 307 - RNA, 21 nt, synthetic construct
  source 1..21: mol_type = other RNA; note = Sense strand of duplex 132
  modified_base order(1,2,3,4,5,6,8,12,14,15,16,17,18,19,20,21): mod_base = OTHER; note = 2'-methoxy modification
  modified_base order(7,9,10,11,13): mod_base = OTHER; note = 2'-fluorinated
  modified_base order(1^2,2^3): mod_base = OTHER; note = Phosphorothioate linkage
tcaggactatctcaagagatt

SEQ ID NO: 308 - RNA, 21 nt, synthetic construct
  source 1..21: mol_type = other RNA; note = Sense strand of duplex 133
  modified_base order(1,2,3,4,5,6,8,12,13,14,15,17,18,19,20,21): mod_base = OTHER; note = 2'-methoxy modification
  modified_base order(7,9,10,11,16): mod_base = OTHER; note = 2'-fluorinated
  modified_base order(1^2,2^3): mod_base = OTHER; note = Phosphorothioate linkage
tcaggactatctcaagagatt

SEQ ID NO: 309 - RNA, 21 nt, synthetic construct
  source 1..21: mol_type = other RNA; note = Sense strand of duplex 134
  modified_base order(1,2,3,4,5,6,8,12,13,14,15,16,18,19,20,21): mod_base = OTHER; note = 2'-methoxy modification
  modified_base order(7,9,10,11,17): mod_base = OTHER; note = 2'-fluorinated
  modified_base order(1^2,2^3): mod_base = OTHER; note = Phosphorothioate linkage
tcaggactatctcaagagatt

SEQ ID NO: 310 - RNA, 21 nt, synthetic construct
  source 1..21: mol_type = other RNA; note = Sense strand of duplex 135/144
  modified_base order(1,2,3,4,5,6,8,12,13,14,15,16,18,19,20,21): mod_base = OTHER; note = 2'-methoxy modification
  modified_base order(7,9,11,17): mod_base = OTHER; note = 2'-fluorinated
  modified_base 10: mod_base = OTHER; note = Deoxynucleotide
  modified_base order(1^2,2^3,20^21): mod_base = OTHER; note = Phosphorothioate linkage
tcaggactatctcaagagatt

SEQ ID NO: 311 - RNA, 21 nt, synthetic construct
  source 1..21: mol_type = other RNA; note = Sense strand of duplex 136
  modified_base order(1,2,3,4,5,6,8,12,13,14,15,16,18,19,20,21): mod_base = OTHER; note = 2'-methoxy modification
  modified_base order(7,10,11,17): mod_base = OTHER; note = 2'-fluorinated
  modified_base 9: mod_base = OTHER; note = Deoxynucleotide
  modified_base order(1^2,2^3,20^21): mod_base = OTHER; note = Phosphorothioate linkage
tcaggactatctcaagagatt

SEQ ID NO: 312 - RNA, 21 nt, synthetic construct
  source 1..21: mol_type = other RNA; note = Sense strand of duplex 137
  modified_base order(1,2,3,4,5,6,8,12,13,14,15,16,18,19,20,21): mod_base = OTHER; note = 2'-methoxy modification
  modified_base order(7,9,10,17): mod_base = OTHER; note = 2'-fluorinated
  modified_base 11: mod_base = OTHER; note = Deoxynucleotide
  modified_base order(1^2,2^3,20^21): mod_base = OTHER; note = Phosphorothioate linkage
tcaggactatctcaagagatt

SEQ ID NO: 313 - RNA, 21 nt, synthetic construct
  source 1..21: mol_type = other RNA; note = Sense strand of duplex 138/148
  modified_base order(1,2,3,4,5,6,7,8,12,13,14,15,16,18,19,20,21): mod_base = OTHER; note = 2'-methoxy modification
  modified_base order(9,10,11,17): mod_base = OTHER; note = 2'-fluorinated
  modified_base order(1^2,2^3,20^21): mod_base = OTHER; note = Phosphorothioate linkage
tcaggactatctcaagagatt

SEQ ID NO: 314 - RNA, 21 nt, synthetic construct
  source 1..21: mol_type = other RNA; note = Sense strand of duplex 139/143
  modified_base order(1,2,3,4,5,6,8,12,13,14,15,16,18,19,20,21): mod_base = OTHER; note = 2'-methoxy modification
  modified_base order(7,9,10,11,17): mod_base = OTHER; note = 2'-fluorinated
  modified_base order(1^2,2^3,20^21): mod_base = OTHER; note = Phosphorothioate linkage
tcaggactatctcaagagatt

SEQ ID NO: 315 - RNA, 21 nt, synthetic construct
  source 1..21: mol_type = other RNA; note = Sense strand of duplex 140/147
  modified_base order(1,2,3,4,5,6,8,12,13,14,15,16,18,19,20,21): mod_base = OTHER; note = 2'-methoxy modification
  modified_base order(7,9,10,11,17): mod_base = OTHER; note = 2'-fluorinated
  modified_base order(1^2,2^3,19^20,20^21): mod_base = OTHER; note = Phosphorothioate linkage
tcaggactatctcaagagatt

SEQ ID NO: 316 - RNA, 21 nt, synthetic construct
  source 1..21: mol_type = other RNA; note = Sense strand of duplex 141
  modified_base order(1,2,3,4,5,6,8,12,13,14,15,18,19,20,21): mod_base = OTHER; note = 2'-methoxy modification
  modified_base order(7,9,10,11,16,17): mod_base = OTHER; note = 2'-fluorinated
  modified_base order(1^2,2^3,20^21): mod_base = OTHER; note = Phosphorothioate linkage
tcaggactatctcaagagatt

SEQ ID NO: 317 - RNA, 21 nt, synthetic construct
  source 1..21: mol_type = other RNA; note = Sense strand of duplex 142/146
  modified_base order(1,2,3,4,5,6,8,12,13,14,16,18,19,20,21): mod_base = OTHER; note = 2'-methoxy modification
  modified_base order(7,9,10,11,15,17): mod_base = OTHER; note = 2'-fluorinated
  modified_base order(1^2,2^3,20^21): mod_base = OTHER; note = Phosphorothioate linkage
tcaggactatctcaagagatt

SEQ ID NO: 318 - RNA, 21 nt, synthetic construct
  source 1..21: mol_type = other RNA; note = Sense strand of duplex 145
  modified_base order(1,2,3,4,5,6,8,12,13,14,15,16,17,18,19,20,21): mod_base = OTHER; note = 2'-methoxy modification
  modified_base order(7,9,11): mod_base = OTHER; note = 2'-fluorinated
  modified_base 10: mod_base = OTHER; note = Deoxynucleotide
  modified_base order(1^2,2^3,20^21): mod_base = OTHER; note = Phosphorothioate linkage
tcaggactatctcaagagatt

SEQ ID NO: 319 - RNA, 21 nt, synthetic construct
  source 1..21: mol_type = other RNA; note = Sense strand of duplex 149/152
  modified_base order(1,2,3,4,5,6,8,10,12,13,14,15,16,17,18,19,20,21): mod_base = OTHER; note = 2'-methoxy modification
  modified_base order(7,9,11): mod_base = OTHER; note = 2'-fluorinated
  modified_base order(1^2,2^3): mod_base = OTHER; note = Phosphorothioate linkage
ctctatgactcagaaacaaaa

SEQ ID NO: 320 - RNA, 21 nt, synthetic construct
  source 1..21: mol_type = other RNA; note = Sense strand of duplex 150/151
  modified_base order(1,2,3,4,5,6,7,8,10,12,14,15,16,17,18,19,20,21): mod_base = OTHER; note = 2'-methoxy modification
  modified_base order(9,11,13): mod_base = OTHER; note = 2'-fluorinated
  modified_base order(1^2,2^3): mod_base = OTHER; note = Phosphorothioate linkage
ctctatgactcagaaacaaaa

SEQ ID NO: 321 - RNA, 21 nt, synthetic construct
  source 1..21: mol_type = other RNA; note = Sense strand of duplex 153
  modified_base order(1,2,3,4,5,6,8,12,13,14,16,17,18,19,20,21): mod_base = OTHER; note = 2'-methoxy modification
  modified_base order(7,9,10,11,15): mod_base = OTHER; note = 2'-fluorinated
  modified_base order(1^2,2^3): mod_base = OTHER; note = Phosphorothioate linkage
ctctatgactcagaaacaaaa

SEQ ID NO: 322 - RNA, 21 nt, synthetic construct
  source 1..21: mol_type = other RNA; note = Sense strand of duplex 154/155
  modified_base order(1,2,3,4,5,6,8,12,13,14,15,16,17,18,19,20,21): mod_base = OTHER; note = 2'-methoxy modification
  modified_base order(7,9,10): mod_base = OTHER; note = 2'-fluorinated
  modified_base 11: mod_base = OTHER; note = Deoxynucleotide
  modified_base order(1^2,2^3): mod_base = OTHER; note = Phosphorothioate linkage
ctctatgactcagaaacaaaa

SEQ ID NO: 323 - RNA, 21 nt, synthetic construct
  source 1..21: mol_type = other RNA; note = Sense strand of duplex 156
  modified_base order(1,2,3,4,5,6,8,12,14,15,16,17,18,19,20,21): mod_base = OTHER; note = 2'-methoxy modification
  modified_base order(7,9,10,11,13): mod_base = OTHER; note = 2'-fluorinated
  modified_base order(1^2,2^3): mod_base = OTHER; note = Phosphorothioate linkage
ctctatgactcagaaacaaaa

SEQ ID NO: 324 - RNA, 21 nt, synthetic construct
  source 1..21: mol_type = other RNA; note = Sense strand of duplex 157
  modified_base order(1,2,3,4,5,6,8,12,13,14,15,17,18,19,20,21): mod_base = OTHER; note = 2'-methoxy modification
  modified_base order(7,9,10,11,16): mod_base = OTHER; note = 2'-fluorinated
  modified_base order(1^2,2^3): mod_base = OTHER; note = Phosphorothioate linkage
ctctatgactcagaaacaaaa

SEQ ID NO: 325 - RNA, 21 nt, synthetic construct
  source 1..21: mol_type = other RNA; note = Sense strand of duplex 158
  modified_base order(1,2,3,4,5,6,8,12,13,14,15,16,18,19,20,21): mod_base = OTHER; note = 2'-methoxy modification
  modified_base order(7,9,10,11,17): mod_base = OTHER; note = 2'-fluorinated
  modified_base order(1^2,2^3): mod_base = OTHER; note = Phosphorothioate linkage
ctctatgactcagaaacaaaa

SEQ ID NO: 326 - RNA, 21 nt, synthetic construct
  source 1..21: mol_type = other RNA; note = Sense strand of duplex 159/168
  modified_base order(1,2,3,4,5,6,8,12,13,14,15,16,18,19,20,21): mod_base = OTHER; note = 2'-methoxy modification
  modified_base order(7,9,11,17): mod_base = OTHER; note = 2'-fluorinated
  modified_base 10: mod_base = OTHER; note = Deoxynucleotide
  modified_base order(1^2,2^3,20^21): mod_base = OTHER; note = Phosphorothioate linkage
ctctatgactcagaaacaaaa

SEQ ID NO: 327 - RNA, 21 nt, synthetic construct
  source 1..21: mol_type = other RNA; note = Sense strand of duplex 160
  modified_base order(1,2,3,4,5,6,8,12,13,14,15,16,18,19,20,21): mod_base = OTHER; note = 2'-methoxy modification
  modified_base order(7,10,11,17): mod_base = OTHER; note = 2'-fluorinated
  modified_base 9: mod_base = OTHER; note = Deoxynucleotide
  modified_base order(1^2,2^3,20^21): mod_base = OTHER; note = Phosphorothioate linkage
ctctatgactcagaaacaaaa

SEQ ID NO: 328 - RNA, 21 nt, synthetic construct
  source 1..21: mol_type = other RNA; note = Sense strand of duplex 161
  modified_base order(1,2,3,4,5,6,8,12,13,14,15,16,18,19,20,21): mod_base = OTHER; note = 2'-methoxy modification
  modified_base order(7,9,10,17): mod_base = OTHER; note = 2'-fluorinated
  modified_base 11: mod_base = OTHER; note = Deoxynucleotide
  modified_base order(1^2,2^3,20^21): mod_base = OTHER; note = Phosphorothioate linkage
ctctatgactcagaaacaaaa

SEQ ID NO: 329 - RNA, 21 nt, synthetic construct
  source 1..21: mol_type = other RNA; note = Sense strand of duplex 162/172
  modified_base order(1,2,3,4,5,6,7,8,12,13,14,15,16,18,19,20,21): mod_base = OTHER; note = 2'-methoxy modification
  modified_base order(9,10,11,17): mod_base = OTHER; note = 2'-fluorinated
  modified_base order(1^2,2^3,20^21): mod_base = OTHER; note = Phosphorothioate linkage
ctctatgactcagaaacaaaa

SEQ ID NO: 330 - RNA, 21 nt, synthetic construct
  source 1..21: mol_type = other RNA; note = Sense strand of duplex 163/167
  modified_base order(1,2,3,4,5,6,8,12,13,14,15,16,18,19,20,21): mod_base = OTHER; note = 2'-methoxy modification
  modified_base order(7,9,10,11,17): mod_base = OTHER; note = 2'-fluorinated
  modified_base order(1^2,2^3,20^21): mod_base = OTHER; note = Phosphorothioate linkage
ctctatgactcagaaacaaaa

SEQ ID NO: 331 - RNA, 21 nt, synthetic construct
  source 1..21: mol_type = other RNA; note = Sense strand of duplex 164/171
  modified_base order(1,2,3,4,5,6,8,12,13,14,15,16,18,19,20,21): mod_base = OTHER; note = 2'-methoxy modification
  modified_base order(7,9,10,11,17): mod_base = OTHER; note = 2'-fluorinated
  modified_base order(1^2,2^3,19^20,20^21): mod_base = OTHER; note = Phosphorothioate linkage
ctctatgactcagaaacaaaa

SEQ ID NO: 332 - RNA, 21 nt, synthetic construct
  source 1..21: mol_type = other RNA; note = Sense strand of duplex 165
  modified_base order(1,2,3,4,5,6,8,12,13,14,15,18,19,20,21): mod_base = OTHER; note = 2'-methoxy modification
  modified_base order(7,9,10,11,16,17): mod_base = OTHER; note = 2'-fluorinated
  modified_base order(1^2,2^3,20^21): mod_base = OTHER; note = Phosphorothioate linkage
ctctatgactcagaaacaaaa

SEQ ID NO: 333 - RNA, 21 nt, synthetic construct
  source 1..21: mol_type = other RNA; note = Sense strand of duplex 166/170
  modified_base order(1,2,3,4,5,6,8,12,13,14,16,18,19,20,21): mod_base = OTHER; note = 2'-methoxy modification
  modified_base order(7,9,10,11,15,17): mod_base = OTHER; note = 2'-fluorinated
  modified_base order(1^2,2^3,20^21): mod_base = OTHER; note = Phosphorothioate linkage
ctctatgactcagaaacaaaa

SEQ ID NO: 334 - RNA, 21 nt, synthetic construct
  source 1..21: mol_type = other RNA; note = Sense strand of duplex 169
  modified_base order(1,2,3,4,5,6,8,12,13,14,15,16,17,18,19,20,21): mod_base = OTHER; note = 2'-methoxy modification
  modified_base order(7,9,11): mod_base = OTHER; note = 2'-fluorinated
  modified_base 10: mod_base = OTHER; note = Deoxynucleotide
  modified_base order(1^2,2^3,20^21): mod_base = OTHER; note = Phosphorothioate linkage
ctctatgactcagaaacaaaa

SEQ ID NO: 335 - RNA, 21 nt, synthetic construct
  source 1..21: mol_type = other RNA; note = Sense strand of duplex 177
  modified_base order(1,2,3,4,5,6,8,12,13,14,16,17,18,19,20,21): mod_base = OTHER; note = 2'-methoxy modification
  modified_base order(7,9,10,11,15): mod_base = OTHER; note = 2'-fluorinated
  modified_base order(1^2,2^3): mod_base = OTHER; note = Phosphorothioate linkage
acagtttagaagccaaactca

SEQ ID NO: 336 - RNA, 21 nt, synthetic construct
  source 1..21: mol_type = other RNA; note = Sense strand of duplex 180
  modified_base order(1,2,3,4,5,6,8,12,14,15,16,17,18,19,20,21): mod_base = OTHER; note = 2'-methoxy modification
  modified_base order(7,9,10,11,13): mod_base = OTHER; note = 2'-fluorinated
  modified_base order(1^2,2^3): mod_base = OTHER; note = Phosphorothioate linkage
acagtttagaagccaaactca

SEQ ID NO: 337 - RNA, 21 nt, synthetic construct
  source 1..21: mol_type = other RNA; note = Sense strand of duplex 181
  modified_base order(1,2,3,4,5,6,8,12,13,14,15,17,18,19,20,21): mod_base = OTHER; note = 2'-methoxy modification
  modified_base order(7,9,10,11,16): mod_base = OTHER; note = 2'-fluorinated
  modified_base order(1^2,2^3): mod_base = OTHER; note = Phosphorothioate linkage
acagtttagaagccaaactca

SEQ ID NO: 338 - RNA, 21 nt, synthetic construct
  source 1..21: mol_type = other RNA; note = Sense strand of duplex 182
  modified_base order(1,2,3,4,5,6,8,12,13,14,15,16,18,19,20,21): mod_base = OTHER; note = 2'-methoxy modification
  modified_base order(7,9,10,11,17): mod_base = OTHER; note = 2'-fluorinated
  modified_base order(1^2,2^3): mod_base = OTHER; note = Phosphorothioate linkage
acagtttagaagccaaactca

SEQ ID NO: 339 - RNA, 21 nt, synthetic construct
  source 1..21: mol_type = other RNA; note = Sense strand of duplex 183
  modified_base order(1,2,3,4,5,6,8,10,12,13,14,15,16,17,18,19,20,21): mod_base = OTHER; note = 2'-methoxy modification
  modified_base order(7,9,11): mod_base = OTHER; note = 2'-fluorinated
  modified_base order(1^2,2^3): mod_base = OTHER; note = Phosphorothioate linkage
cagtttagaagccaaactcaa

SEQ ID NO: 340 - RNA, 21 nt, synthetic construct
  source 1..21: mol_type = other RNA; note = Sense strand of duplex 184/185
  modified_base order(1,2,3,4,5,6,7,8,10,12,14,15,16,17,18,19,20,21): mod_base = OTHER; note = 2'-methoxy modification
  modified_base order(9,11,13): mod_base = OTHER; note = 2'-fluorinated
  modified_base order(1^2,2^3): mod_base = OTHER; note = Phosphorothioate linkage
cagtttagaagccaaactcaa

SEQ ID NO: 341 - RNA, 21 nt, synthetic construct
  source 1..21: mol_type = other RNA; note = Sense strand of duplex 187
  modified_base order(1,2,3,4,5,6,8,12,13,14,16,17,18,19,20,21): mod_base = OTHER; note = 2'-methoxy modification
  modified_base order(7,9,10,11,15): mod_base = OTHER; note = 2'-fluorinated
  modified_base order(1^2,2^3): mod_base = OTHER; note = Phosphorothioate linkage
cagtttagaagccaaactcaa

SEQ ID NO: 342 - RNA, 21 nt, synthetic construct
  source 1..21: mol_type = other RNA; note = Sense strand of duplex 188/191
  modified_base order(1,2,3,4,5,6,8,10,12,13,14,15,16,17,18,19,20,21): mod_base = OTHER; note = 2'-methoxy modification
  modified_base order(7,9,11): mod_base = OTHER; note = 2'-fluorinated
  modified_base order(1^2,2^3): mod_base = OTHER; note = Phosphorothioate linkage
atcgattagtgtcaaaggctt

SEQ ID NO: 343 - RNA, 21 nt, synthetic construct
  source 1..21: mol_type = other RNA; note = Sense strand of duplex 189/190
  modified_base order(1,2,3,4,5,6,7,8,10,12,14,15,16,17,18,19,20,21): mod_base = OTHER; note = 2'-methoxy modification
  modified_base order(9,11,13): mod_base = OTHER; note = 2'-fluorinated
  modified_base order(1^2,2^3): mod_base = OTHER; note = Phosphorothioate linkage
atcgattagtgtcaaaggctt

SEQ ID NO: 344 - RNA, 21 nt, synthetic construct
  source 1..21: mol_type = other RNA; note = Sense strand of duplex 192
  modified_base order(1,2,3,4,5,6,8,12,13,14,16,17,18,19,20,21): mod_base = OTHER; note = 2'-methoxy modification
  modified_base order(7,9,10,11,15): mod_base = OTHER; note = 2'-fluorinated
  modified_base order(1^2,2^3): mod_base = OTHER; note = Phosphorothioate linkage
atcgattagtgtcaaaggctt

SEQ ID NO: 345 - RNA, 21 nt, synthetic construct
  source 1..21: mol_type = other RNA; note = Sense strand of duplex 193/194
  modified_base order(1,2,3,4,5,6,8,12,13,14,15,16,17,18,19,20,21): mod_base = OTHER; note = 2'-methoxy modification
  modified_base order(7,9,10): mod_base = OTHER; note = 2'-fluorinated
  modified_base 11: mod_base = OTHER; note = Deoxynucleotide
  modified_base order(1^2,2^3): mod_base = OTHER; note = Phosphorothioate linkage
atcgattagtgtcaaaggctt

SEQ ID NO: 346 - RNA, 21 nt, synthetic construct
  source 1..21: mol_type = other RNA; note = Sense strand of duplex 195
  modified_base order(1,2,3,4,5,6,8,12,14,15,16,17,18,19,20,21): mod_base = OTHER; note = 2'-methoxy modification
  modified_base order(7,9,10,11,13): mod_base = OTHER; note = 2'-fluorinated
  modified_base order(1^2,2^3): mod_base = OTHER; note = Phosphorothioate linkage
atcgattagtgtcaaaggctt

SEQ ID NO: 347 - RNA, 21 nt, synthetic construct
  source 1..21: mol_type = other RNA; note = Sense strand of duplex 196
  modified_base order(1,2,3,4,5,6,8,12,13,14,15,17,18,19,20,21): mod_base = OTHER; note = 2'-methoxy modification
  modified_base order(7,9,10,11,16): mod_base = OTHER; note = 2'-fluorinated
  modified_base order(1^2,2^3): mod_base = OTHER; note = Phosphorothioate linkage
atcgattagtgtcaaaggctt

SEQ ID NO: 348 - RNA, 21 nt, synthetic construct
  source 1..21: mol_type = other RNA; note = Sense strand of duplex 197
  modified_base order(1,2,3,4,5,6,8,12,13,14,15,16,18,19,20,21): mod_base = OTHER; note = 2'-methoxy modification
  modified_base order(7,9,10,11,17): mod_base = OTHER; note = 2'-fluorinated
  modified_base order(1^2,2^3): mod_base = OTHER; note = Phosphorothioate linkage
atcgattagtgtcaaaggctt

SEQ ID NO: 349 - RNA, 21 nt, synthetic construct
  source 1..21: mol_type = other RNA; note = Sense strand of duplex 198/201
  modified_base order(1,2,3,4,5,6,8,10,12,13,14,15,16,17,18,19,20,21): mod_base = OTHER; note = 2'-methoxy modification
  modified_base order(7,9,11): mod_base = OTHER; note = 2'-fluorinated
  modified_base order(1^2,2^3): mod_base = OTHER; note = Phosphorothioate linkage
gtgtcaaaggctttaaacata

SEQ ID NO: 350 - RNA, 21 nt, synthetic construct
  source 1..21: mol_type = other RNA; note = Sense strand of duplex 199/200
  modified_base order(1,2,3,4,5,6,7,8,10,12,14,15,16,17,18,19,20,21): mod_base = OTHER; note = 2'-methoxy modification
  modified_base order(9,11,13): mod_base = OTHER; note = 2'-fluorinated
  modified_base order(1^2,2^3): mod_base = OTHER; note = Phosphorothioate linkage
gtgtcaaaggctttaaacata

SEQ ID NO: 351 - RNA, 21 nt, synthetic construct
  source 1..21: mol_type = other RNA; note = Sense strand of duplex 202
  modified_base order(1,2,3,4,5,6,8,12,13,14,16,17,18,19,20,21): mod_base = OTHER; note = 2'-methoxy modification
  modified_base order(7,9,10,11,15): mod_base = OTHER; note = 2'-fluorinated
  modified_base order(1^2,2^3): mod_base = OTHER; note = Phosphorothioate linkage
gtgtcaaaggctttaaacata

SEQ ID NO: 352 - RNA, 21 nt, synthetic construct
  source 1..21: mol_type = other RNA; note = Sense strand of duplex 203/204
  modified_base order(1,2,3,4,5,6,8,12,13,14,15,16,17,18,19,20,21): mod_base = OTHER; note = 2'-methoxy modification
  modified_base order(7,9,10): mod_base = OTHER; note = 2'-fluorinated
  modified_base 11: mod_base = OTHER; note = Deoxynucleotide
  modified_base order(1^2,2^3): mod_base = OTHER; note = Phosphorothioate linkage
gtgtcaaaggctttaaacata

SEQ ID NO: 353 - RNA, 21 nt, synthetic construct
  source 1..21: mol_type = other RNA; note = Sense strand of duplex 205
  modified_base order(1,2,3,4,5,6,8,12,14,15,16,17,18,19,20,21): mod_base = OTHER; note = 2'-methoxy modification
  modified_base order(7,9,10,11,13): mod_base = OTHER; note = 2'-fluorinated
  modified_base order(1^2,2^3): mod_base = OTHER; note = Phosphorothioate linkage
gtgtcaaaggctttaaacata

SEQ ID NO: 354 - RNA, 21 nt, synthetic construct
  source 1..21: mol_type = other RNA; note = Sense strand of duplex 206
  modified_base order(1,2,3,4,5,6,8,12,13,14,15,17,18,19,20,21): mod_base = OTHER; note = 2'-methoxy modification
  modified_base order(7,9,10,11,16): mod_base = OTHER; note = 2'-fluorinated
  modified_base order(1^2,2^3): mod_base = OTHER; note = Phosphorothioate linkage
gtgtcaaaggctttaaacata

SEQ ID NO: 355 - RNA, 21 nt, synthetic construct
  source 1..21: mol_type = other RNA; note = Sense strand of duplex 207
  modified_base order(1,2,3,4,5,6,8,12,13,14,15,16,18,19,20,21): mod_base = OTHER; note = 2'-methoxy modification
  modified_base order(7,9,10,11,17): mod_base = OTHER; note = 2'-fluorinated
  modified_base order(1^2,2^3): mod_base = OTHER; note = Phosphorothioate linkage
gtgtcaaaggctttaaacata

SEQ ID NO: 356 - RNA, 21 nt, synthetic construct
  source 1..21: mol_type = other RNA; note = Sense strand of duplex 208
  modified_base order(1,2,3,4,5,6,8,10,12,13,14,15,16,17,18,19,20,21): mod_base = OTHER; note = 2'-methoxy modification
  modified_base order(7,9,11): mod_base = OTHER; note = 2'-fluorinated
  modified_base order(1^2,2^3,19^20,20^21): mod_base = OTHER; note = Phosphorothioate linkage
gtgtcaaaggctttaaacata

SEQ ID NO: 357 - RNA, 21 nt, synthetic construct
  source 1..21: mol_type = other RNA; note = Sense strand of duplex 209
  modified_base order(1,2,3,4,5,6,7,8,10,12,14,15,16,17,18,19,20,21): mod_base = OTHER; note = 2'-methoxy modification
  modified_base order(9,11,13): mod_base = OTHER; note = 2'-fluorinated
  modified_base order(1^2,2^3,19^20,20^21): mod_base = OTHER; note = Phosphorothioate linkage
gtgtcaaaggctttaaacata

SEQ ID NO: 358 - RNA, 21 nt, synthetic construct
  source 1..21: mol_type = other RNA; note = Sense strand of duplex 210
  modified_base order(1,2,3,4,5,6,8,12,13,14,15,16,17,18,19,20,21): mod_base = OTHER; note = 2'-methoxy modification
  modified_base order(7,9,10): mod_base = OTHER; note = 2'-fluorinated
  modified_base 11: mod_base = OTHER; note = Deoxynucleotide
  modified_base order(1^2,2^3,19^20,20^21): mod_base = OTHER; note = Phosphorothioate linkage
gtgtcaaaggctttaaacata

SEQ ID NO: 359 - RNA, 21 nt, synthetic construct
  source 1..21: mol_type = other RNA; note = Sense strand of duplex 211
  modified_base order(1,2,3,4,5,6,8,12,13,14,15,16,17,18,19,20,21): mod_base = OTHER; note = 2'-methoxy modification
  modified_base order(7,9,11): mod_base = OTHER; note = 2'-fluorinated
  modified_base 10: mod_base = OTHER; note = Deoxynucleotide
  modified_base order(1^2,2^3,19^20,20^21): mod_base = OTHER; note = Phosphorothioate linkage
gtgtcaaaggctttaaacata

SEQ ID NO: 360 - RNA, 21 nt, synthetic construct
  source 1..21: mol_type = other RNA; note = Sense strand of duplex 212
  modified_base order(1,2,3,4,5,6,8,12,13,14,15,16,18,19,20,21): mod_base = OTHER; note = 2'-methoxy modification
  modified_base order(7,9,10,11,17): mod_base = OTHER; note = 2'-fluorinated
  modified_base order(1^2,2^3,19^20,20^21): mod_base = OTHER; note = Phosphorothioate linkage
gtgtcaaaggctttaaacata

SEQ ID NO: 361 - RNA, 21 nt, synthetic construct
  source 1..21: mol_type = other RNA; note = Sense strand of duplex 213
  modified_base order(1,2,3,4,5,6,8,10,12,13,14,15,16,17,18,19,20,21): mod_base = OTHER; note = 2'-methoxy modification
  modified_base order(7,9,11): mod_base = OTHER; note = 2'-fluorinated
  modified_base 21: mod_base = OTHER; note = Inverted abasic residue
  modified_base order(1^2,2^3,>21): mod_base = OTHER; note = Phosphorothioate linkage
gtgtcaaaggctttaaacata

SEQ ID NO: 362 - RNA, 21 nt, synthetic construct
  source 1..21: mol_type = other RNA; note = Sense strand of duplex 214
  modified_base order(1,2,3,4,5,6,7,8,10,12,14,15,16,17,18,19,20,21): mod_base = OTHER; note = 2'-methoxy modification
  modified_base order(9,11,13): mod_base = OTHER; note = 2'-fluorinated
  modified_base 21: mod_base = OTHER; note = Inverted abasic residue
  modified_base order(1^2,2^3,>21): mod_base = OTHER; note = Phosphorothioate linkage
gtgtcaaaggctttaaacata

SEQ ID NO: 363 - RNA, 21 nt, synthetic construct
  source 1..21: mol_type = other RNA; note = Sense strand of duplex 215
  modified_base order(1,2,3,4,5,6,8,12,13,14,15,16,17,18,19,20,21): mod_base = OTHER; note = 2'-methoxy modification
  modified_base order(7,9,10): mod_base = OTHER; note = 2'-fluorinated
  modified_base 11: mod_base = OTHER; note = Deoxynucleotide
  modified_base 21: mod_base = OTHER; note = Inverted abasic residue
  modified_base order(1^2,2^3,>21): mod_base = OTHER; note = Phosphorothioate linkage
gtgtcaaaggctttaaacata

SEQ ID NO: 364 - RNA, 21 nt, synthetic construct
  source 1..21: mol_type = other RNA; note = Sense strand of duplex 216
  modified_base order(1,2,3,4,5,6,8,12,13,14,15,16,17,18,19,20,21): mod_base = OTHER; note = 2'-methoxy modification
  modified_base order(7,9,11): mod_base = OTHER; note = 2'-fluorinated
  modified_base 10: mod_base = OTHER; note = Deoxynucleotide
  modified_base 21: mod_base = OTHER; note = Inverted abasic residue
  modified_base order(1^2,2^3,>21): mod_base = OTHER; note = Phosphorothioate linkage
gtgtcaaaggctttaaacata

SEQ ID NO: 365 - RNA, 21 nt, synthetic construct
  source 1..21: mol_type = other RNA; note = Sense strand of duplex 217
  modified_base order(1,2,3,4,5,6,8,12,13,14,15,16,18,19,20,21): mod_base = OTHER; note = 2'-methoxy modification
  modified_base order(7,9,10,11,17): mod_base = OTHER; note = 2'-fluorinated
  modified_base 21: mod_base = OTHER; note = Inverted abasic residue
  modified_base order(1^2,2^3,>21): mod_base = OTHER; note = Phosphorothioate linkage
gtgtcaaaggctttaaacata

SEQ ID NO: 366 - RNA, 21 nt, synthetic construct
  source 1..21: mol_type = other RNA; note = Sense strand of duplex 218/221
  modified_base order(1,2,3,4,5,6,8,10,12,13,14,15,16,17,18,19,20,21): mod_base = OTHER; note = 2'-methoxy modification
  modified_base order(7,9,11): mod_base = OTHER; note = 2'-fluorinated
  modified_base order(1^2,2^3): mod_base = OTHER; note = Phosphorothioate linkage
tcggaggagatgctcacttca

SEQ ID NO: 367 - RNA, 21 nt, synthetic construct
  source 1..21: mol_type = other RNA; note = Sense strand of duplex 219/220
  modified_base order(1,2,3,4,5,6,7,8,10,12,14,15,16,17,18,19,20,21): mod_base = OTHER; note = 2'-methoxy modification
  modified_base order(9,11,13): mod_base = OTHER; note = 2'-fluorinated
  modified_base order(1^2,2^3): mod_base = OTHER; note = Phosphorothioate linkage
tcggaggagatgctcacttca

SEQ ID NO: 368 - RNA, 21 nt, synthetic construct
  source 1..21: mol_type = other RNA; note = Sense strand of duplex 222
  modified_base order(1,2,3,4,5,6,8,12,13,14,16,17,18,19,20,21): mod_base = OTHER; note = 2'-methoxy modification
  modified_base order(7,9,10,11,15): mod_base = OTHER; note = 2'-fluorinated
  modified_base order(1^2,2^3): mod_base = OTHER; note = Phosphorothioate linkage
tcggaggagatgctcacttca

SEQ ID NO: 369 - RNA, 21 nt, synthetic construct
  source 1..21: mol_type = other RNA; note = Sense strand of duplex 223/224
  modified_base order(1,2,3,4,5,6,8,12,13,14,15,16,17,18,19,20,21): mod_base = OTHER; note = 2'-methoxy modification
  modified_base order(7,9,10): mod_base = OTHER; note = 2'-fluorinated
  modified_base 11: mod_base = OTHER; note = Deoxynucleotide
  modified_base order(1^2,2^3): mod_base = OTHER; note = Phosphorothioate linkage
tcggaggagatgctcacttca

SEQ ID NO: 370 - RNA, 21 nt, synthetic construct
  source 1..21: mol_type = other RNA; note = Sense strand of duplex 225
  modified_base order(1,2,3,4,5,6,8,12,14,15,16,17,18,19,20,21): mod_base = OTHER; note = 2'-methoxy modification
  modified_base order(7,9,10,11,13): mod_base = OTHER; note = 2'-fluorinated
  modified_base order(1^2,2^3): mod_base = OTHER; note = Phosphorothioate linkage
tcggaggagatgctcacttca

SEQ ID NO: 371 - RNA, 21 nt, synthetic construct
  source 1..21: mol_type = other RNA; note = Sense strand of duplex 226
  modified_base order(1,2,3,4,5,6,8,12,13,14,15,17,18,19,20,21): mod_base = OTHER; note = 2'-methoxy modification
  modified_base order(7,9,10,11,16): mod_base = OTHER; note = 2'-fluorinated
  modified_base order(1^2,2^3): mod_base = OTHER; note = Phosphorothioate linkage
tcggaggagatgctcacttca

SEQ ID NO: 372 - RNA, 21 nt, synthetic construct
  source 1..21: mol_type = other RNA; note = Sense strand of duplex 227
  modified_base order(1,2,3,4,5,6,8,12,13,14,15,16,18,19,20,21): mod_base = OTHER; note = 2'-methoxy modification
  modified_base order(7,9,10,11,17): mod_base = OTHER; note = 2'-fluorinated
  modified_base order(1^2,2^3): mod_base = OTHER; note = Phosphorothioate linkage
tcggaggagatgctcacttca

SEQ ID NO: 373 - RNA, 21 nt, synthetic construct
  source 1..21: mol_type = other RNA; note = Sense strand of duplex 228/231
  modified_base order(1,2,3,4,5,6,8,10,12,13,14,15,16,17,18,19,20,21): mod_base = OTHER; note = 2'-methoxy modification
  modified_base order(7,9,11): mod_base = OTHER; note = 2'-fluorinated
  modified_base order(1^2,2^3): mod_base = OTHER; note = Phosphorothioate linkage
ttcgatgaggatgaacgctga

SEQ ID NO: 374 - RNA, 21 nt, synthetic construct
  source 1..21: mol_type = other RNA; note = Sense strand of duplex 229/230
  modified_base order(1,2,3,4,5,6,7,8,10,12,14,15,16,17,18,19,20,21): mod_base = OTHER; note = 2'-methoxy modification
  modified_base order(9,11,13): mod_base = OTHER; note = 2'-fluorinated
  modified_base order(1^2,2^3): mod_base = OTHER; note = Phosphorothioate linkage
ttcgatgaggatgaacgctga

SEQ ID NO: 375 - RNA, 21 nt, synthetic construct
  source 1..21: mol_type = other RNA; note = Sense strand of duplex 232
  modified_base order(1,2,3,4,5,6,8,12,13,14,16,17,18,19,20,21): mod_base = OTHER; note = 2'-methoxy modification
  modified_base order(7,9,10,11,15): mod_base = OTHER; note = 2'-fluorinated
  modified_base order(1^2,2^3): mod_base = OTHER; note = Phosphorothioate linkage
ttcgatgaggatgaacgctga

SEQ ID NO: 376 - RNA, 21 nt, synthetic construct
  source 1..21: mol_type = other RNA; note = Sense strand of duplex 233/234
  modified_base order(1,2,3,4,5,6,8,12,13,14,15,16,17,18,19,20,21): mod_base = OTHER; note = 2'-methoxy modification
  modified_base order(7,9,10): mod_base = OTHER; note = 2'-fluorinated
  modified_base 11: mod_base = OTHER; note = Deoxynucleotide
  modified_base order(1^2,2^3): mod_base = OTHER; note = Phosphorothioate linkage
ttcgatgaggatgaacgctga

SEQ ID NO: 377 - RNA, 21 nt, synthetic construct
  source 1..21: mol_type = other RNA; note = Sense strand of duplex 235
  modified_base order(1,2,3,4,5,6,8,12,14,15,16,17,18,19,20,21): mod_base = OTHER; note = 2'-methoxy modification
  modified_base order(7,9,10,11,13): mod_base = OTHER; note = 2'-fluorinated
  modified_base order(1^2,2^3): mod_base = OTHER; note = Phosphorothioate linkage
ttcgatgaggatgaacgctga

SEQ ID NO: 378 - RNA, 21 nt, synthetic construct
  source 1..21: mol_type = other RNA; note = Sense strand of duplex 236
  modified_base order(1,2,3,4,5,6,8,12,13,14,15,17,18,19,20,21): mod_base = OTHER; note = 2'-methoxy modification
  modified_base order(7,9,10,11,16): mod_base = OTHER; note = 2'-fluorinated
  modified_base order(1^2,2^3): mod_base = OTHER; note = Phosphorothioate linkage
ttcgatgaggatgaacgctga

SEQ ID NO: 379 - RNA, 21 nt, synthetic construct
  source 1..21: mol_type = other RNA; note = Sense strand of duplex 237
  modified_base order(1,2,3,4,5,6,8,12,13,14,15,16,18,19,20,21): mod_base = OTHER; note = 2'-methoxy modification
  modified_base order(7,9,10,11,17): mod_base = OTHER; note = 2'-fluorinated
  modified_base order(1^2,2^3): mod_base = OTHER; note = Phosphorothioate linkage
ttcgatgaggatgaacgctga

SEQ ID NO: 380-416 - skipped (37 entries)